European Patent Application EP 4 549 586 A2, published May 7, 2025. Title: Treatment And Inhibition Of Inflammatory Lung Diseases In Patients Having Risk Alleles In The Genes Encoding IL33 And IL1RL1. Applicant: Regeneron Pharmaceuticals, Inc. Application EP, filed March 20, 2018. The sequence listing filed with the application follows.

SEQUENCE LISTING (358 sequences)

SEQ ID NO: 1 - DNA, 366 bp, synthetic construct
  misc_feature 1..366: note = Synthetic
  source 1..366: mol_type = other DNA
caggtgcagctggtggagtctgggggaggcgtggtccagcctgggaggtccctgagactctcctgtgcagcgtctggattcaccttcagtagttatggcatgcattgggtccgccaggctccaggcaaggggctggagtgggtggcagttatatggtatgatggaagaaataaatactatacagactccgtgaagggccgattcaccatctccagagacaattccaagaacacgctgtatctgcaaatggacagcctgagagccgaggacacggctgtgtattactgtgcgagagagaggtatatcagcagctattatggggggttcgacccctggggccagggagccctggtcaccgtctcctca

SEQ ID NO: 2 - protein, 122 aa, synthetic construct
  REGION 1..122: note = Synthetic
QVQLVESGGGVVQPGRSLRLSCAASGFTFSSYGMHWVRQAPGKGLEWVAVIWYDGRNKYYTDSVKGRFTISRDNSKNTLYLQMDSLRAEDTAVYYCARERYISSYYGGFDPWGQGALVTVSS

SEQ ID NO: 3 - DNA, 24 bp, synthetic construct
  misc_feature 1..24: note = Synthetic
  source 1..24: mol_type = other DNA
ggattcaccttcagtagttatggc

SEQ ID NO: 4 - protein, 8 aa, synthetic construct
  REGION 1..8: note = Synthetic
GFTFSSYG

SEQ ID NO: 5 - DNA, 24 bp, synthetic construct
  misc_feature 1..24: note = Synthetic
  source 1..24: mol_type = other DNA
atatggtatgatggaagaaataaa

SEQ ID NO: 6 - protein, 8 aa, synthetic construct
  REGION 1..8: note = Synthetic
IWYDGRNK

SEQ ID NO: 7 - DNA, 45 bp, synthetic construct
  misc_feature 1..45: note = Synthetic
  source 1..45: mol_type = other DNA
gcgagagagaggtatatcagcagctattatggggggttcgacccc

SEQ ID NO: 8 - protein, 15 aa, synthetic construct
  REGION 1..15: note = Synthetic
ARERYISSYYGGFDP

SEQ ID NO: 9 - DNA, 321 bp, synthetic construct
  misc_feature 1..321: note = Synthetic
  source 1..321: mol_type = other DNA
gacatccagatgacccagtctccatcctccgtgtctgcatctgtaggagacagagtcaccatcacttgtcgggcgagtcagggtattagtagttggttagcctggtatcagcagaaaccagggaaagcccctaaggtcctgatctatgctgcatccagtttgcaaagtggggtcccatcaaggttcagcggcagtggatctgggacagatttcactctcaccatcagcagcctgcagcctgaagattttgcaacttactattgtcaacaggctaacagtttcccattcactttcggccctgggaccaaactggatatcaag

SEQ ID NO: 10 - protein, 107 aa, synthetic construct
  REGION 1..107: note = Synthetic
DIQMTQSPSSVSASVGDRVTITCRASQGISSWLAWYQQKPGKAPKVLIYAASSLQSGVPSRFSGSGSGTDFTLTISSLQPEDFATYYCQQANSFPFTFGPGTKLDIK

SEQ ID NO: 11 - DNA, 18 bp, synthetic construct
  misc_feature 1..18: note = Synthetic
  source 1..18: mol_type = other DNA
cagggtattagtagttgg

SEQ ID NO: 12 - protein, 6 aa, synthetic construct
  REGION 1..6: note = Synthetic
QGISSW

SEQ ID NO: 13-14 - skipped (2 entries)

SEQ ID NO: 15 - DNA, 27 bp, synthetic construct
  misc_feature 1..27: note = Synthetic
  source 1..27: mol_type = other DNA
caacaggctaacagtttcccattcact

SEQ ID NO: 16 - protein, 9 aa, synthetic construct
  REGION 1..9: note = Synthetic
QQANSFPFT

SEQ ID NO: 17 - DNA, 357 bp, synthetic construct
  misc_feature 1..357: note = Synthetic
  source 1..357: mol_type = other DNA
gaggtgcagctgttggagtctgggggagacttggtacagcctggggggtccctgagactctcctgtgcagcctctggattcaccttcagcagctatgccatgagctgggtccgccaggctccagggaaggggctggagtgggtctcagttattagtggtagtggaagtagcacagactacgcagactccgtgaagggccggttcaccatttccagagacaattccagggacacgctgcatctgcaaatgaacagcctgagagccgaggacacggccgtatattactgtgcgaaaacgttctactacttctacggtttggacgtctggggccaagggaccacggtcaccgtctcctca

SEQ ID NO: 18 - protein, 119 aa, synthetic construct
  REGION 1..119: note = Synthetic
EVQLLESGGDLVQPGGSLRLSCAASGFTFSSYAMSWVRQAPGKGLEWVSVISGSGSSTDYADSVKGRFTISRDNSRDTLHLQMNSLRAEDTAVYYCAKTFYYFYGLDVWGQGTTVTVSS

SEQ ID NO: 19 - DNA, 24 bp, synthetic construct
  misc_feature 1..24: note = Synthetic
  source 1..24: mol_type = other DNA
ggattcaccttcagcagctatgcc

SEQ ID NO: 20 - protein, 8 aa, synthetic construct
  REGION 1..8: note = Synthetic
GFTFSSYA

SEQ ID NO: 21 - DNA, 24 bp, synthetic construct
  misc_feature 1..24: note = Synthetic
  source 1..24: mol_type = other DNA
attagtggtagtggaagtagcaca

SEQ ID NO: 22 - protein, 8 aa, synthetic construct
  REGION 1..8: note = Synthetic
ISGSGSST

SEQ ID NO: 23 - DNA, 36 bp, synthetic construct
  misc_feature 1..36: note = Synthetic
  source 1..36: mol_type = other DNA
gcgaaaacgttctactacttctacggtttggacgtc

SEQ ID NO: 24 - protein, 12 aa, synthetic construct
  REGION 1..12: note = Synthetic
AKTFYYFYGLDV

SEQ ID NO: 25 - DNA, 321 bp, synthetic construct
  misc_feature 1..321: note = Synthetic
  source 1..321: mol_type = other DNA
gacatccagatgacccagtctccatcctccctgtctgcatctttaagagacagagtcaccatcacttgccgggcgagtcagggcattagcaattatttagcctggtatcagcagaaaccagggaaagttcctaaggtcctaatctatgctgcatccactttgcaatcaggggtcccatctcggttcagtggcagtggatctgggacagttttcactctcaccatcagcagcctgcagactgaagatgttgcaacttattactgtcaaaagtatagcagtgccccattcactttcggccctgggaccaaagtggatatcaaa

SEQ ID NO: 26 - protein, 107 aa, synthetic construct
  REGION 1..107: note = Synthetic
DIQMTQSPSSLSASLRDRVTITCRASQGISNYLAWYQQKPGKVPKVLIYAASTLQSGVPSRFSGSGSGTVFTLTISSLQTEDVATYYCQKYSSAPFTFGPGTKVDIK

SEQ ID NO: 27 - DNA, 18 bp, synthetic construct
  misc_feature 1..18: note = Synthetic
  source 1..18: mol_type = other DNA
cagggcattagcaattat

SEQ ID NO: 28 - protein, 6 aa, synthetic construct
  REGION 1..6: note = Synthetic
QGISNY

SEQ ID NO: 29-30 - skipped (2 entries)

SEQ ID NO: 31 - DNA, 27 bp, synthetic construct
  misc_feature 1..27: note = Synthetic
  source 1..27: mol_type = other DNA
caaaagtatagcagtgccccattcact

SEQ ID NO: 32 - protein, 9 aa, synthetic construct
  REGION 1..9: note = Synthetic
QKYSSAPFT

SEQ ID NO: 33 - DNA, 351 bp, synthetic construct
  misc_feature 1..351: note = Synthetic
  source 1..351: mol_type = other DNA
caggtgcttctggtacagtctggggctgaggtgaagaagcctggggccacagtgaaggtctcctgcaaggcttctggatccactttcaccggctactatatgcactgggtgcgacaggcccctggacaagggcttgagtggatgggatggatcaaccctaacaatggtggcacaaactatgcacagaagtttcagggcagggtcaccatgaccagggacacgtccatcagcacagcctacatggaattgagcaggctgagatctgacgacacggccgtatattactgtgcgagagagttgcggtataactggaagtcctggggccagggaaccctggtcaccgtctcctca

SEQ ID NO: 34 - protein, 117 aa, synthetic construct
  REGION 1..117: note = Synthetic
QVLLVQSGAEVKKPGATVKVSCKASGSTFTGYYMHWVRQAPGQGLEWMGWINPNNGGTNYAQKFQGRVTMTRDTSISTAYMELSRLRSDDTAVYYCARELRYNWKSWGQGTLVTVSS

SEQ ID NO: 35 - DNA, 24 bp, synthetic construct
  misc_feature 1..24: note = Synthetic
  source 1..24: mol_type = other DNA
ggatccactttcaccggctactat

SEQ ID NO: 36 - protein, 8 aa, synthetic construct
  REGION 1..8: note = Synthetic
GSTFTGYY

SEQ ID NO: 37 - DNA, 24 bp, synthetic construct
  misc_feature 1..24: note = Synthetic
  source 1..24: mol_type = other DNA
atcaaccctaacaatggtggcaca

SEQ ID NO: 38 - protein, 8 aa, synthetic construct
  REGION 1..8: note = Synthetic
INPNNGGT

SEQ ID NO: 39 - DNA, 30 bp, synthetic construct
  misc_feature 1..30: note = Synthetic
  source 1..30: mol_type = other DNA
gcgagagagttgcggtataactggaagtcc

SEQ ID NO: 40 - protein, 10 aa, synthetic construct
  REGION 1..10: note = Synthetic
ARELRYNWKS

SEQ ID NO: 41 - DNA, 324 bp, synthetic construct
  misc_feature 1..324: note = Synthetic
  source 1..324: mol_type = other DNA
gaaattgtgttgacgcagtctccaggcaccctgtctttgtctccaggggaaagagtcaccctctcctgcagggccagtcagagtgttggcaggccctacttagcctggtaccaacagatacctggccaggctcccaggctcctcatctatggtgcatccagcagggccactgacatcccagacaggttcagtggcaatgggtctgggacagacttcactctcaccatcagtagactggagcctgaagattttgcagtgtattactgtcagcagtatgataattccccttatacttttggccaggggaccaggctggagatcaaa

SEQ ID NO: 42 - protein, 108 aa, synthetic construct
  REGION 1..108: note = Synthetic
EIVLTQSPGTLSLSPGERVTLSCRASQSVGRPYLAWYQQIPGQAPRLLIYGASSRATDIPDRFSGNGSGTDFTLTISRLEPEDFAVYYCQQYDNSPYTFGQGTRLEIK

SEQ ID NO: 43 - DNA, 21 bp, synthetic construct
  misc_feature 1..21: note = Synthetic
  source 1..21: mol_type = other DNA
cagagtgttggcaggccctac

SEQ ID NO: 44 - protein, 7 aa, synthetic construct
  REGION 1..7: note = Synthetic
QSVGRPY

SEQ ID NO: 45-46 - skipped (2 entries)

SEQ ID NO: 47 - DNA, 27 bp, synthetic construct
  misc_feature 1..27: note = Synthetic
  source 1..27: mol_type = other DNA
cagcagtatgataattccccttatact

SEQ ID NO: 48 - protein, 9 aa, synthetic construct
  REGION 1..9: note = Synthetic
QQYDNSPYT

SEQ ID NO: 49 - DNA, 366 bp, synthetic construct
  misc_feature 1..366: note = Synthetic
  source 1..366: mol_type = other DNA
gaggtgcagctggtggagtctgggggaggcttggtacaacctggggggtccctgagactctcctgtgcagcctctggattcacctttagaagctttgccatgagctgggtccgccaggctccagggaaggggctggaattggtctcagatctcaggactagtggtggtagtacatactacgcagactccgtgaagggccggctcaccatctccagagacaattccaagaacacgctgtatctgcaaatgaacagcctgagagccgaggacacggccgtatattactgtgcgaaaagccactatagcaccagctggttcgggggctttgactactggggccagggaaccctggtcactgtctcctca

SEQ ID NO: 50 - protein, 122 aa, synthetic construct
  REGION 1..122: note = Synthetic
EVQLVESGGGLVQPGGSLRLSCAASGFTFRSFAMSWVRQAPGKGLELVSDLRTSGGSTYYADSVKGRLTISRDNSKNTLYLQMNSLRAEDTAVYYCAKSHYSTSWFGGFDYWGQGTLVTVSS

SEQ ID NO: 51 - DNA, 24 bp, synthetic construct
  misc_feature 1..24: note = Synthetic
  source 1..24: mol_type = other DNA
ggattcacctttagaagctttgcc

SEQ ID NO: 52 - protein, 8 aa, synthetic construct
  REGION 1..8: note = Synthetic
GFTFRSFA

SEQ ID NO: 53 - DNA, 24 bp, synthetic construct
  misc_feature 1..24: note = Synthetic
  source 1..24: mol_type = other DNA
ctcaggactagtggtggtagtaca

SEQ ID NO: 54 - protein, 8 aa, synthetic construct
  REGION 1..8: note = Synthetic
LRTSGGST

SEQ ID NO: 55 - DNA, 45 bp, synthetic construct
  misc_feature 1..45: note = Synthetic
  source 1..45: mol_type = other DNA
gcgaaaagccactatagcaccagctggttcgggggctttgactac

SEQ ID NO: 56 - protein, 15 aa, synthetic construct
  REGION 1..15: note = Synthetic
AKSHYSTSWFGGFDY

SEQ ID NO: 57 - DNA, 321 bp, synthetic construct
  misc_feature 1..321: note = Synthetic
  source 1..321: mol_type = other DNA
gacatccagatgacccagtctccatcttccgtgtctgcttctgtaggagacagagtcaccatcacttgtcgggcgagtcagggttttagcagctggttagcctggtatcagcagaaaccagggaaagcccctaagctcctgatctatgctgcatccagtttgcaaagtggggtcccatcaaggttcagcggcagtggatctgggacagatttcactctcaccatcaccaacctgcagcctgaagattttgcaacttactattgtcaacaggctaacagtttccctctcactttcggcggagggaccaaggtggagatcaaa

SEQ ID NO: 58 - protein, 107 aa, synthetic construct
  REGION 1..107: note = Synthetic
DIQMTQSPSSVSASVGDRVTITCRASQGFSSWLAWYQQKPGKAPKLLIYAASSLQSGVPSRFSGSGSGTDFTLTITNLQPEDFATYYCQQANSFPLTFGGGTKVEIK

SEQ ID NO: 59 - DNA, 18 bp, synthetic construct
  misc_feature 1..18: note = Synthetic
  source 1..18: mol_type = other DNA
cagggttttagcagctgg

SEQ ID NO: 60 - protein, 6 aa, synthetic construct
  REGION 1..6: note = Synthetic
QGFSSW

SEQ ID NO: 61-62 - skipped (2 entries)

SEQ ID NO: 63 - DNA, 27 bp, synthetic construct
  misc_feature 1..27: note = Synthetic
  source 1..27: mol_type = other DNA
caacaggctaacagtttccctctcact

SEQ ID NO: 64 - protein, 9 aa, synthetic construct
  REGION 1..9: note = Synthetic
QQANSFPLT

SEQ ID NO: 65 - DNA, 366 bp, synthetic construct
  misc_feature 1..366: note = Synthetic
  source 1..366: mol_type = other DNA
gaggtgcagctggtggagtctgggggaggcttggtacagcctggggggtccctgagactctcctgtgcagcctctggattcacgtttagcagctatgtcatgagctgggtccgccaggctccagggaaggggctggagtgggtctcaagtattagtggtaatggtggtagcacaaactacgcagactccgtgaagggccggttcaccatctccagagacaattccaagaacacgctgtttctggaaatgaacagcctgagagccgaggacacggccgtatattactgtgcgaaatcactgggaactaccacgacttttttggggtttgactattggggccagggaaccctggtcaccgtctcctca

SEQ ID NO: 66 - protein, 122 aa, synthetic construct
  REGION 1..122: note = Synthetic
EVQLVESGGGLVQPGGSLRLSCAASGFTFSSYVMSWVRQAPGKGLEWVSSISGNGGSTNYADSVKGRFTISRDNSKNTLFLEMNSLRAEDTAVYYCAKSLGTTTTFLGFDYWGQGTLVTVSS

SEQ ID NO: 67 - DNA, 24 bp, synthetic construct
  misc_feature 1..24: note = Synthetic
  source 1..24: mol_type = other DNA
ggattcacgtttagcagctatgtc

SEQ ID NO: 68 - protein, 8 aa, synthetic construct
  REGION 1..8: note = Synthetic
GFTFSSYV

SEQ ID NO: 69 - DNA, 24 bp, synthetic construct
  misc_feature 1..24: note = Synthetic
  source 1..24: mol_type = other DNA
attagtggtaatggtggtagcaca

SEQ ID NO: 70 - protein, 8 aa, synthetic construct
  REGION 1..8: note = Synthetic
ISGNGGST

SEQ ID NO: 71 - DNA, 45 bp, synthetic construct
  misc_feature 1..45: note = Synthetic
  source 1..45: mol_type = other DNA
gcgaaatcactgggaactaccacgacttttttggggtttgactat

SEQ ID NO: 72 - protein, 15 aa, synthetic construct
  REGION 1..15: note = Synthetic
AKSLGTTTTFLGFDY

SEQ ID NO: 73 - DNA, 321 bp, synthetic construct
  misc_feature 1..321: note = Synthetic
  source 1..321: mol_type = other DNA
gacatccagatgacccagtctccatcttccgtgtctgcatctgtaggagacagagtcaccatcacttgtcgggcgagtcagggtattagcagctggttagcctggtatcagcagaaaccagggaaagcccctaaactcctgatctatgctgcatccagtttgcaaagtggggtcccatcaaggttcagcggcagtggatctgggacatatttcactctcaccatcagcagcctgcagcctgaagattttgcaacttactattgtcaacaggctaacagtttccctctcactttcggcggagggaccaaggtggagatcaaa

SEQ ID NO: 74 - protein, 107 aa, synthetic construct
  REGION 1..107: note = Synthetic
DIQMTQSPSSVSASVGDRVTITCRASQGISSWLAWYQQKPGKAPKLLIYAASSLQSGVPSRFSGSGSGTYFTLTISSLQPEDFATYYCQQANSFPLTFGGGTKVEIK

SEQ ID NO: 75 - DNA, 18 bp, synthetic construct
  misc_feature 1..18: note = Synthetic
  source 1..18: mol_type = other DNA
cagggtattagcagctgg

SEQ ID NO: 76 - protein, 6 aa, synthetic construct
  REGION 1..6: note = Synthetic
QGISSW

SEQ ID NO: 77-78 - skipped (2 entries)

SEQ ID NO: 79 - DNA, 27 bp, synthetic construct
  misc_feature 1..27: note = Synthetic
  source 1..27: mol_type = other DNA
caacaggctaacagtttccctctcact

SEQ ID NO: 80 - protein, 9 aa, synthetic construct
  REGION 1..9: note = Synthetic
QQANSFPLT

SEQ ID NO: 81 - DNA, 363 bp, synthetic construct
  misc_feature 1..363: note = Synthetic
  source 1..363: mol_type = other DNA
caggtgcagctgcaggagtcgggcccaggactggtgaagccttcggagaccctgtccctcacctgcactgtctctggtggctccatcagtagttattactggagctggatccggcagcccccagggaagggactggagttgattgggtatatttattacagtgggagcaccaattataacccctccctcaagagtcgagtcaccatatctgtagacacgtccaagaaccacttctccctgaagctgagctctgtgaccgctgcggacacggccgtatattactgtgcgagatcccagtataccagtagttggtacggttcttttgatatctggggccaagggacaatggtcaccgtctcttca

SEQ ID NO: 82 - protein, 121 aa, synthetic construct
  REGION 1..121: note = Synthetic
QVQLQESGPGLVKPSETLSLTCTVSGGSISSYYWSWIRQPPGKGLELIGYIYYSGSTNYNPSLKSRVTISVDTSKNHFSLKLSSVTAADTAVYYCARSQYTSSWYGSFDIWGQGTMVTVSS

SEQ ID NO: 83 - DNA, 24 bp, synthetic construct
  misc_feature 1..24: note = Synthetic
  source 1..24: mol_type = other DNA
ggtggctccatcagtagttattac

SEQ ID NO: 84 - protein, 8 aa, synthetic construct
  REGION 1..8: note = Synthetic
GGSISSYY

SEQ ID NO: 85 - DNA, 21 bp, synthetic construct
  misc_feature 1..21: note = Synthetic
  source 1..21: mol_type = other DNA
atttattacagtgggagcacc

SEQ ID NO: 86 - protein, 7 aa, synthetic construct
  REGION 1..7: note = Synthetic
IYYSGST

SEQ ID NO: 87 - DNA, 45 bp, synthetic construct
  misc_feature 1..45: note = Synthetic
  source 1..45: mol_type = other DNA
gcgagatcccagtataccagtagttggtacggttcttttgatatc

SEQ ID NO: 88 - protein, 15 aa, synthetic construct
  REGION 1..15: note = Synthetic
ARSQYTSSWYGSFDI

SEQ ID NO: 89 - DNA, 321 bp, synthetic construct
  misc_feature 1..321: note = Synthetic
  source 1..321: mol_type = other DNA
gacatccagatgacccagtctccatcttccgtgtctgcatctgtaggagacagagtcaccatcacttgtcgggcgagtcagggtattagcacctggttagcctggtttcagcagaaaccagggaaagcccctaagctcctgatctatgctgcatccactttacaaggtggggtcccatcaaggttcagcggcagtggatctgggccagaattcactctcaccatcagcagcctgcagcctgaagattttgcaacttactattgtcaacaggctaacagtttcccgtggacgttcggccaagggaccaaggtggaaatcaaa

SEQ ID NO: 90 - protein, 107 aa, synthetic construct
  REGION 1..107: note = Synthetic
DIQMTQSPSSVSASVGDRVTITCRASQGISTWLAWFQQKPGKAPKLLIYAASTLQGGVPSRFSGSGSGPEFTLTISSLQPEDFATYYCQQANSFPWTFGQGTKVEIK

SEQ ID NO: 91 - DNA, 18 bp, synthetic construct
  misc_feature 1..18: note = Synthetic
  source 1..18: mol_type = other DNA
cagggtattagcacctgg

SEQ ID NO: 92 - protein, 6 aa, synthetic construct
  REGION 1..6: note = Synthetic
QGISTW

SEQ ID NO: 93-94 - skipped (2 entries)

SEQ ID NO: 95 - DNA, 27 bp, synthetic construct
  misc_feature 1..27: note = Synthetic
  source 1..27: mol_type = other DNA
caacaggctaacagtttcccgtggacg

SEQ ID NO: 96 - protein, 9 aa, synthetic construct
  REGION 1..9: note = Synthetic
QQANSFPWT

SEQ ID NO: 97 - DNA, 366 bp, synthetic construct
  misc_feature 1..366: note = Synthetic
  source 1..366: mol_type = other DNA
caggttcagctggtgcagtctggagctgaggtgaagaagcctggggcctcagtgaaggtctcctgcaaggcctctggttacacctttaacagctatggtatcagctgggtgcgacaggcccctggacaagggcttgagtggatgggatggatcagctcccacaatggtaacagtcactatgtacagaagttccagggcagagtctccatgaccacagacacatccacgagtacagcctacatggaactgaggagccttagatctgacgacacggccgtgtattactgtgcgagacactcgtataccaccagctggtacgggggttttgactattggggccagggaaccctggtcaccgtctcctca

SEQ ID NO: 98 - protein, 122 aa, synthetic construct
  REGION 1..122: note = Synthetic
QVQLVQSGAEVKKPGASVKVSCKASGYTFNSYGISWVRQAPGQGLEWMGWISSHNGNSHYVQKFQGRVSMTTDTSTSTAYMELRSLRSDDTAVYYCARHSYTTSWYGGFDYWGQGTLVTVSS

SEQ ID NO: 99 - DNA, 24 bp, synthetic construct
  misc_feature 1..24: note = Synthetic
  source 1..24: mol_type = other DNA
ggttacacctttaacagctatggt

SEQ ID NO: 100 - protein, 8 aa, synthetic construct
  REGION 1..8: note = Synthetic
GYTFNSYG

SEQ ID NO: 101 - DNA, 24 bp, synthetic construct
  misc_feature 1..24: note = Synthetic
  source 1..24: mol_type = other DNA
atcagctcccacaatggtaacagt

SEQ ID NO: 102 - protein, 8 aa, synthetic construct
  REGION 1..8: note = Synthetic
ISSHNGNS

SEQ ID NO: 103 - DNA, 45 bp, synthetic construct
  misc_feature 1..45: note = Synthetic
  source 1..45: mol_type = other DNA
gcgagacactcgtataccaccagctggtacgggggttttgactat

SEQ ID NO: 104 - protein, 15 aa, synthetic construct
  REGION 1..15: note = Synthetic
ARHSYTTSWYGGFDY

SEQ ID NO: 105 - DNA, 321 bp, synthetic construct
  misc_feature 1..321: note = Synthetic
  source 1..321: mol_type = other DNA
gacatccagatgacccagtctccatcttccgtgtctgcatctgtaggagacagagtcaccatcacttgtcgggcgagtcagggttttagcagctggttagcctggtatcagcagaaaccagggaaagcccctcagctcctgatctatgctgcatccagtttgcaaagtggggtcccatcaaggttcagcggcagtggatctgggtcagatttcactctcaccatcagcagcctgcagcctgaagattttgcaacttactattgtcaacaggctaacagtttccctctcactttcggcggagggaccaaggtggagatcaaa

SEQ ID NO: 106 - protein, 107 aa, synthetic construct
  REGION 1..107: note = Synthetic
DIQMTQSPSSVSASVGDRVTITCRASQGFSSWLAWYQQKPGKAPQLLIYAASSLQSGVPSRFSGSGSGSDFTLTISSLQPEDFATYYCQQANSFPLTFGGGTKVEIK

SEQ ID NO: 107 - DNA, 18 bp, synthetic construct
  misc_feature 1..18: note = Synthetic
  source 1..18: mol_type = other DNA
cagggttttagcagctgg

SEQ ID NO: 108 - protein, 6 aa, synthetic construct
  REGION 1..6: note = Synthetic
QGFSSW

SEQ ID NO: 109-110 - skipped (2 entries)

SEQ ID NO: 111 - DNA, 27 bp, synthetic construct
  misc_feature 1..27: note = Synthetic
  source 1..27: mol_type = other DNA
caacaggctaacagtttccctctcact

SEQ ID NO: 112 - protein, 9 aa, synthetic construct
  REGION 1..9: note = Synthetic
QQANSFPLT

SEQ ID NO: 113 - DNA, 366 bp, synthetic construct
  misc_feature 1..366: note = Synthetic
  source 1..366: mol_type = other DNA
gaggtgcagctggtggagtccgggggaggcttggttcagccgggggggtccctgagactctcctgtgcagcctctggaatcaccttgagcagctatggcatgagctgggtccgccaggctccagggaagggactggagtgggtcgcatccatttttggtagtggtggtggcccatactacgcagactccgtgaagggccggttcaccatgtccagagacaattccaagaacacgctgtatttgcaaatgaacagcctgagagccgaggacacggccgtatattattgtgcgaaagatcgatacagtgggagctactacggaggttttgactactggggccggggaaccctggtcaccgtctcctca

SEQ ID NO: 114 - protein, 122 aa, synthetic construct
  REGION 1..122: note = Synthetic
EVQLVESGGGLVQPGGSLRLSCAASGITLSSYGMSWVRQAPGKGLEWVASIFGSGGGPYYADSVKGRFTMSRDNSKNTLYLQMNSLRAEDTAVYYCAKDRYSGSYYGGFDYWGRGTLVTVSS

SEQ ID NO: 115 - DNA, 24 bp, synthetic construct
  misc_feature 1..24: note = Synthetic
  source 1..24: mol_type = other DNA
ggaatcaccttgagcagctatggc

SEQ ID NO: 116 - protein, 8 aa, synthetic construct
  REGION 1..8: note = Synthetic
GITLSSYG

SEQ ID NO: 117 - DNA, 24 bp, synthetic construct
  misc_feature 1..24: note = Synthetic
  source 1..24: mol_type = other DNA
atttttggtagtggtggtggccca

SEQ ID NO: 118 - protein, 8 aa, synthetic construct
  REGION 1..8: note = Synthetic
IFGSGGGP

SEQ ID NO: 119 - DNA, 45 bp, synthetic construct
  misc_feature 1..45: note = Synthetic
  source 1..45: mol_type = other DNA
gcgaaagatcgatacagtgggagctactacggaggttttgactac

SEQ ID NO: 120 - protein, 15 aa, synthetic construct
  REGION 1..15: note = Synthetic
AKDRYSGSYYGGFDY

SEQ ID NO: 121 - DNA, 321 bp, synthetic construct
  misc_feature 1..321: note = Synthetic
  source 1..321: mol_type = other DNA
gacatccagatgacccagtctccatcttccgtgtctgcatctgtaggagacagagtcaccatcacttgtcgggcgagtcagggtattaccagctggttagcctggtatcagcagaaaccagggaaagcccctacactcctgatctatgctgcatccagtttgcaaactggggtcccatcaaggttcagcggcagtggatctgggacagatttcactctcaccatcagcagcctgcagcctgaacattttgcaacttactattgtcaacaggctaacagtttccctcctactttcggcggagggaccaaggtggagatcaaa

SEQ ID NO: 122 - protein, 107 aa, synthetic construct
  REGION 1..107: note = Synthetic
DIQMTQSPSSVSASVGDRVTITCRASQGITSWLAWYQQKPGKAPTLLIYAASSLQTGVPSRFSGSGSGTDFTLTISSLQPEHFATYYCQQANSFPPTFGGGTKVEIK

SEQ ID NO: 123 - DNA, 18 bp, synthetic construct
  misc_feature 1..18: note = Synthetic
  source 1..18: mol_type = other DNA
cagggtattaccagctgg

SEQ ID NO: 124 - protein, 6 aa, synthetic construct
  REGION 1..6: note = Synthetic
QGITSW

SEQ ID NO: 125-126 - skipped (2 entries)

SEQ ID NO: 127 - DNA, 27 bp, synthetic construct
  misc_feature 1..27: note = Synthetic
  source 1..27: mol_type = other DNA
caacaggctaacagtttccctcctact

SEQ ID NO: 128 - protein, 9 aa, synthetic construct
  REGION 1..9: note = Synthetic
QQANSFPPT

SEQ ID NO: 129 - DNA, 366 bp, synthetic construct
  misc_feature 1..366: note = Synthetic
  source 1..366: mol_type = other DNA
gaggtgcagctggtggagtctgggggaggcttggtacagcctggggggtccctaagactctcctgtgcagcctctggattcacctttagcagttatgccttgacctgggtccgccaggctccagggaaggggctggagtgggtctcttttattagtggtagtggtggtaggccattctacgcagactccgtgaagggccggttcaccatctccagagacaattccaagaacatgctgtatctgcaaatgaacagcctgagagccgaggacacggccatatattactgtgcgaagtccctgtataccaccagctggtacggggggttcgactcctggggccagggaaccctggtcaccgtctcctca

SEQ ID NO: 130 - protein, 122 aa, synthetic construct
  REGION 1..122: note = Synthetic
EVQLVESGGGLVQPGGSLRLSCAASGFTFSSYALTWVRQAPGKGLEWVSFISGSGGRPFYADSVKGRFTISRDNSKNMLYLQMNSLRAEDTAIYYCAKSLYTTSWYGGFDSWGQGTLVTVSS

SEQ ID NO: 131 - DNA, 24 bp, synthetic construct
  misc_feature 1..24: note = Synthetic
  source 1..24: mol_type = other DNA
ggattcacctttagcagttatgcc

SEQ ID NO: 132 - protein, 8 aa, synthetic construct
  REGION 1..8: note = Synthetic
GFTFSSYA

SEQ ID NO: 133 - DNA, 24 bp, synthetic construct
  misc_feature 1..24: note = Synthetic
  source 1..24: mol_type = other DNA
attagtggtagtggtggtaggcca

SEQ ID NO: 134 - protein, 8 aa, synthetic construct
  REGION 1..8: note = Synthetic
ISGSGGRP

SEQ ID NO: 135 - DNA, 45 bp, synthetic construct
  misc_feature 1..45: note = Synthetic
  source 1..45: mol_type = other DNA
gcgaagtccctgtataccaccagctggtacggggggttcgactcc

SEQ ID NO: 136 - protein, 15 aa, synthetic construct
  REGION 1..15: note = Synthetic
AKSLYTTSWYGGFDS

SEQ ID NO: 137 - DNA, 321 bp, synthetic construct
  misc_feature 1..321: note = Synthetic
  source 1..321: mol_type = other DNA
gacatccagatgacccagtctccatcttccgtgtctgcatctgtaggagacagagtcaccatcacttgtcgggcgagtcagggtgtcgtcagctggttagcctggtatcagcagaaaccagggaaagcccctaagctcctgatctatgctgcatccagtttgcaaagtggggtcccatcaaggttcagcggcagtggatctgggacagatttcactctcaccatcagcagcctgcagcctgaagattttgcaacttattattgtcaacagtctaacagtttccctttcactctcggccctgggaccaaagtggatatcaaa

SEQ ID NO: 138 - protein, 107 aa, synthetic construct
  REGION 1..107: note = Synthetic
DIQMTQSPSSVSASVGDRVTITCRASQGVVSWLAWYQQKPGKAPKLLIYAASSLQSGVPSRFSGSGSGTDFTLTISSLQPEDFATYYCQQSNSFPFTLGPGTKVDIK

SEQ ID NO: 139 - DNA, 18 bp, synthetic construct
  misc_feature 1..18: note = Synthetic
  source 1..18: mol_type = other DNA
cagggtgtcgtcagctgg

SEQ ID NO: 140 - protein, 6 aa, synthetic construct
  REGION 1..6: note = Synthetic
QGVVSW

SEQ ID NO: 141-142 - skipped (2 entries)

SEQ ID NO: 143 - DNA, 24 bp, synthetic construct
  misc_feature 1..24: note = Synthetic
  source 1..24: mol_type = other DNA
caacagtctaacagtttccctttc

SEQ ID NO: 144 - protein, 8 aa, synthetic construct
  REGION 1..8: note = Synthetic
QQSNSFPF

SEQ ID NO: 145 - DNA, 366 bp, synthetic construct
  misc_feature 1..366: note = Synthetic
  source 1..366: mol_type = other DNA
caggtgcagctggtgcagtctggggctgaagtgaagaagcctggggcctcagtgaaggtctcctgcaaggcttctggatacaccttcaccggccactatatgtactggatgcgacaggcccctggacaagggcttgagtggatgggatggatcaaccctaacagtggtggcacaaactatgcacagaagtttcaggacagggtcaccatgaccagggacacgtccatcagcacagcctacatggagctgagcaggctgagatctgacgacacggccgtgtattactgtgcgagagggagatatggcagtagctggtacggggggtttgagtactggggccagggaaccctggtcaccgtctcctca

SEQ ID NO: 146 - protein, 122 aa, synthetic construct
  REGION 1..122: note = Synthetic
QVQLVQSGAEVKKPGASVKVSCKASGYTFTGHYMYWMRQAPGQGLEWMGWINPNSGGTNYAQKFQDRVTMTRDTSISTAYMELSRLRSDDTAVYYCARGRYGSSWYGGFEYWGQGTLVTVSS

SEQ ID NO: 147 - DNA, 24 bp, synthetic construct
  misc_feature 1..24: note = Synthetic
  source 1..24: mol_type = other DNA
ggatacaccttcaccggccactat

SEQ ID NO: 148 - protein, 8 aa, synthetic construct
  REGION 1..8: note = Synthetic
GYTFTGHY

SEQ ID NO: 149 - DNA, 24 bp, synthetic construct
  misc_feature 1..24: note = Synthetic
  source 1..24: mol_type = other DNA
atcaaccctaacagtggtggcaca

SEQ ID NO: 150 - protein, 8 aa, synthetic construct
  REGION 1..8: note = Synthetic
INPNSGGT

SEQ ID NO: 151 - DNA, 45 bp, synthetic construct
  misc_feature 1..45: note = Synthetic
  source 1..45: mol_type = other DNA
gcgagagggagatatggcagtagctggtacggggggtttgagtac

SEQ ID NO: 152 - protein, 15 aa, synthetic construct
  REGION 1..15: note = Synthetic
ARGRYGSSWYGGFEY

SEQ ID NO: 153 - DNA, 321 bp, synthetic construct
  misc_feature 1..321: note = Synthetic
  source 1..321: mol_type = other DNA
gacatccagatgacccagtctccatcttccgtgtctgcatctgttggagacagagtcaccatcacttgtcgggcgagtcagggtattaccagctggttagcctggtatcagcagaaaccagggaaagcccctaacctcctgatctatgctgcagccagtttacaaagtggggtcccatcaaggttcagcggcagtggatctgggacggatttcactctcaccatcagcagcctgcagcctgaagactttacaacttactattgtcaacaggcttacagtctccctctcactttcggcggagggaccaaggtggagatcaaa

SEQ ID NO: 154 - protein, 107 aa, synthetic construct
  REGION 1..107: note = Synthetic
DIQMTQSPSSVSASVGDRVTITCRASQGITSWLAWYQQKPGKAPNLLIYAAASLQSGVPSRFSGSGSGTDFTLTISSLQPEDFTTYYCQQAYSLPLTFGGGTKVEIK

SEQ ID NO: 155 - DNA, 18 bp, synthetic construct
  misc_feature 1..18: note = Synthetic
  source 1..18: mol_type = other DNA
cagggtattaccagctgg

SEQ ID NO: 156 - protein, 6 aa, synthetic construct
  REGION 1..6: note = Synthetic
QGITSW

SEQ ID NO: 157-158 - skipped (2 entries)

SEQ ID NO: 159 - DNA, 27 bp, synthetic construct
  misc_feature 1..27: note = Synthetic
  source 1..27: mol_type = other DNA
caacaggcttacagtctccctctcact

SEQ ID NO: 160 - protein, 9 aa, synthetic construct
  REGION 1..9: note = Synthetic
QQAYSLPLT

SEQ ID NO: 161 - DNA, 366 bp, synthetic construct
  misc_feature 1..366: note = Synthetic
  source 1..366: mol_type = other DNA
caggtgcagctggtggagtctgggggaggcgtggtccagcctgggaggtccctgagactctcctgtgcagcctctggattcaccttcagtagctatggcttgcactgggtccgccagtctccaggcaaggggctggaatgggtggcacttatatcatatgacggaagtaataaatactatgcagactccgtgaagggccgattcaccatctccagagacaattccaagaacacgctgtatctgcaaatgaacagcctgagacctgaggacacggctggatatttctgtgcgaaatccctatatacaaccagctggtacgggggctttgactattggggccagggaaccctggtcaccgtctcctca

SEQ ID NO: 162 - protein, 122 aa, synthetic construct
  REGION 1..122: note = Synthetic
QVQLVESGGGVVQPGRSLRLSCAASGFTFSSYGLHWVRQSPGKGLEWVALISYDGSNKYYADSVKGRFTISRDNSKNTLYLQMNSLRPEDTAGYFCAKSLYTTSWYGGFDYWGQGTLVTVSS

SEQ ID NO: 163 - DNA, 24 bp, synthetic construct
  misc_feature 1..24: note = Synthetic
  source 1..24: mol_type = other DNA
ggattcaccttcagtagctatggc

SEQ ID NO: 164 - protein, 8 aa, synthetic construct
  REGION 1..8: note = Synthetic
GFTFSSYG

SEQ ID NO: 165 - DNA, 24 bp, synthetic construct
  misc_feature 1..24: note = Synthetic
  source 1..24: mol_type = other DNA
atatcatatgacggaagtaataaa

SEQ ID NO: 166 - protein, 8 aa, synthetic construct
  REGION 1..8: note = Synthetic
ISYDGSNK

SEQ ID NO: 167 - DNA, 45 bp, synthetic construct
  misc_feature 1..45: note = Synthetic
  source 1..45: mol_type = other DNA
gcgaaatccctatatacaaccagctggtacgggggctttgactat

SEQ ID NO: 168 - protein, 15 aa, synthetic construct
  REGION 1..15: note = Synthetic
AKSLYTTSWYGGFDY

SEQ ID NO: 169 - DNA, 321 bp, synthetic construct
  misc_feature 1..321: note = Synthetic
  source 1..321: mol_type = other DNA
gacatccagatgacccagtctccatcttccgtgtctgcatctgtaggagacagagtcaccatcacttgtcgggcgagtcagggtattagaagctggttagcctggtatcagcaaaaaccagggaaagcccctaacctcctgatctatgctgcgtccagtttgcaaagtggggtcccatcaaggttcagcggcagtggatctgggacagatttcactctcaccatcagcagcctgcagcctgaagattttgcaacttactattgtcaacaggctaacagtttccctcccactttcggccctgggaccaaagtggatatcaaa

SEQ ID NO: 170 - protein, 107 aa, synthetic construct
  REGION 1..107: note = Synthetic
DIQMTQSPSSVSASVGDRVTITCRASQGIRSWLAWYQQKPGKAPNLLIYAASSLQSGVPSRFSGSGSGTDFTLTISSLQPEDFATYYCQQANSFPPTFGPGTKVDIK

SEQ ID NO: 171 - DNA, 18 bp, synthetic construct
  misc_feature 1..18: note = Synthetic
  source 1..18: mol_type = other DNA
cagggtattagaagctgg

SEQ ID NO: 172 - protein, 6 aa, synthetic construct
  REGION 1..6: note = Synthetic
QGIRSW

SEQ ID NO: 173-174 - skipped (2 entries)

SEQ ID NO: 175 - DNA, 27 bp, synthetic construct
  misc_feature 1..27: note = Synthetic
  source 1..27: mol_type = other DNA
caacaggctaacagtttccctcccact

SEQ ID NO: 176 - protein, 9 aa, synthetic construct
  REGION 1..9: note = Synthetic
QQANSFPPT

SEQ ID NO: 177 - DNA, 366 bp, synthetic construct
  misc_feature 1..366: note = Synthetic
  source 1..366: mol_type = other DNA
gaggtgcagctggtggagtctgggggaggcttggtacagcctggggggtccctgagactctcctgtgcagcctctgggttcaccttcagcaactatgccatgacctgggtccgccaggctccagggaaggggctggagtgggtctcaactatcagtggcagtggtgataacacatactacgcagactccgtgcagggccggttcaccatctccagaggccattccaagaacacgctgtatctgcaaatgaacagcctgagagccgaggacacggccgtatattactgtgcgaaacctacgtatagcagaagctggtacggtgcttttgatttctggggccaagggacaatggtcaccgtctcttca

SEQ ID NO: 178 - protein, 122 aa, synthetic construct
  REGION 1..122: note = Synthetic
EVQLVESGGGLVQPGGSLRLSCAASGFTFSNYAMTWVRQAPGKGLEWVSTISGSGDNTYYADSVQGRFTISRGHSKNTLYLQMNSLRAEDTAVYYCAKPTYSRSWYGAFDFWGQGTMVTVSS

SEQ ID NO: 179 - DNA, 24 bp, synthetic construct
  misc_feature 1..24: note = Synthetic
  source 1..24: mol_type = other DNA
gggttcaccttcagcaactatgcc

SEQ ID NO: 180 - protein, 8 aa, synthetic construct
  REGION 1..8: note = Synthetic
GFTFSNYA

SEQ ID NO: 181 - DNA, 24 bp, synthetic construct
  misc_feature 1..24: note = Synthetic
  source 1..24: mol_type = other DNA
atcagtggcagtggtgataacaca

SEQ ID NO: 182 - protein, 8 aa, synthetic construct
  REGION 1..8: note = Synthetic
ISGSGDNT

SEQ ID NO: 183 - DNA, 45 bp, synthetic construct
  misc_feature 1..45: note = Synthetic
  source 1..45: mol_type = other DNA
gcgaaacctacgtatagcagaagctggtacggtgcttttgatttc

SEQ ID NO: 184 - protein, 15 aa, synthetic construct
  REGION 1..15: note = Synthetic
AKPTYSRSWYGAFDF

SEQ ID NO: 185 - DNA, 321 bp, synthetic construct
  misc_feature 1..321: note = Synthetic
  source 1..321: mol_type = other DNA
gacatccagatgacccagtctccatcctccgtgtctgcatctgtaggagacagagtcaccatcacttgtcgggcgagtcagggtattagcagctggttagcctggtatcagcagaaaccggggaaagcccctcaactcctgatctatgctgcatccagattgcaaagtggggtcccatcaaggttctggggcagtggatctgggacagatttcactctcaccatcagcagcctgcagcctgaagattttgcaacttactattgtcaacaggctaacaatttcccattcactttcggccctgggaccaaagtggatatcaaa

SEQ ID NO: 186 - protein, 107 aa, synthetic construct
  REGION 1..107: note = Synthetic
DIQMTQSPSSVSASVGDRVTITCRASQGISSWLAWYQQKPGKAPQLLIYAASRLQSGVPSRFWGSGSGTDFTLTISSLQPEDFATYYCQQANNFPFTFGPGTKVDIK

SEQ ID NO: 187 - DNA, 18 bp, synthetic construct
  misc_feature 1..18: note = Synthetic
  source 1..18: mol_type = other DNA
cagggtattagcagctgg

SEQ ID NO: 188 - protein, 6 aa, synthetic construct
  REGION 1..6: note = Synthetic
QGISSW

SEQ ID NO: 189-190 - skipped (2 entries)

SEQ ID NO: 191 - DNA, 27 bp, synthetic construct
  misc_feature 1..27: note = Synthetic
  source 1..27: mol_type = other DNA
caacaggctaacaatttcccattcact

SEQ ID NO: 192 - protein, 9 aa, synthetic construct
  REGION 1..9: note = Synthetic
QQANNFPFT

SEQ ID NO: 193 - DNA, 366 bp, synthetic construct
  misc_feature 1..366: note = Synthetic
  source 1..366: mol_type = other DNA
caggttcagctggtgcagtctggagctgaggtgaagaagcctggggcctcagtgaaggtctcctgcaaggcttctggttacacctttaccagttatggtatcagctgggtgcgacaggcccctggacaaggccttgagtggatgggatggatccgcgcttacaatggttacacaaactatgcacagaagtttcagggcagagtcaccatgaccacagacacatccacgaacaccgcctacatggagctgaggaccctgaattctgacgatacggccgtttattactgtgcgagagatcgatatagtgggagcttccacggtaactttgactactggggccagggaaccctggtcaccgtctcctca

SEQ ID NO: 194 - protein, 122 aa, synthetic construct
  REGION 1..122: note = Synthetic
QVQLVQSGAEVKKPGASVKVSCKASGYTFTSYGISWVRQAPGQGLEWMGWIRAYNGYTNYAQKFQGRVTMTTDTSTNTAYMELRTLNSDDTAVYYCARDRYSGSFHGNFDYWGQGTLVTVSS

SEQ ID NO: 195 - DNA, 24 bp, synthetic construct
  misc_feature 1..24: note = Synthetic
  source 1..24: mol_type = other DNA
ggttacacctttaccagttatggt

SEQ ID NO: 196 - protein, 8 aa, synthetic construct
  REGION 1..8: note = Synthetic
GYTFTSYG

SEQ ID NO: 197 - DNA, 24 bp, synthetic construct
  misc_feature 1..24: note = Synthetic
  source 1..24: mol_type = other DNA
atccgcgcttacaatggttacaca

SEQ ID NO: 198 - protein, 8 aa, synthetic construct
  REGION 1..8: note = Synthetic
IRAYNGYT

SEQ ID NO: 199 - DNA, 45 bp, synthetic construct
  misc_feature 1..45: note = Synthetic
  source 1..45: mol_type = other DNA
gcgagagatcgatatagtgggagcttccacggtaactttgactac

SEQ ID NO: 200 - protein, 15 aa, synthetic construct
  REGION 1..15: note = Synthetic
ARDRYSGSFHGNFDY

SEQ ID NO: 201 - DNA, 321 bp, synthetic construct
  misc_feature 1..321: note = Synthetic
  source 1..321: mol_type = other DNA
gacatccagatgacccagtctccatcttccgtgtctgcgtctgtaggagacagagtgaccatcacttgtcgggcgagtcagggtattttcagctggttagcctggtatcagcagaaaccagggaaagcccctaaggtcctaatctatgctgcatccaatttggaaagtggggtcccatcaaggttcagcggcagtggatctgggacagatttcactctcaccatcagcagcctgcagcctgaagattttgcaacttactattgtcaacaggctaacagtttaccgctcactttcggcggagggaccaaggtggagatcaaa

SEQ ID NO: 202 - protein, 107 aa, synthetic construct
  REGION 1..107: note = Synthetic
DIQMTQSPSSVSASVGDRVTITCRASQGIFSWLAWYQQKPGKAPKVLIYAASNLESGVPSRFSGSGSGTDFTLTISSLQPEDFATYYCQQANSLPLTFGGGTKVEIK

SEQ ID NO: 203 - DNA, 18 bp, synthetic construct
  misc_feature 1..18: note = Synthetic
  source 1..18: mol_type = other DNA
cagggtattttcagctgg

SEQ ID NO: 204 - protein, 6 aa, synthetic construct
  REGION 1..6: note = Synthetic
QGIFSW

SEQ ID NO: 205-206 - skipped (2 entries)

SEQ ID NO: 207 - DNA, 27 bp, synthetic construct
  misc_feature 1..27: note = Synthetic
  source 1..27: mol_type = other DNA
caacaggctaacagtttaccgctcact

SEQ ID NO: 208 - protein, 9 aa, synthetic construct
  REGION 1..9: note = Synthetic
QQANSLPLT

SEQ ID NO: 209 - DNA, 366 bp, synthetic construct
  misc_feature 1..366: note = Synthetic
  source 1..366: mol_type = other DNA
gaggtgcagctggtggagtctgggggaggcttggtccagcctggggggtccctgagactctcctgtgcagcctctggattcaccttcagtacctattctatgcactgggtccgccaggctccagggaagggactggaatatgtttcaactattaataataatggggataccacatattatgcagactctgtgaagggcagattcaccatctccagagacaattccaagaacacgctgtatcttcaactgggcagcctgagacctgaggacatggctgtgtattactgtgcgagacagacgtataccagcagctggtacggggggttcgactcctggggccagggaaccctggtcaccgtctcctca

SEQ ID NO: 210 - protein, 122 aa, synthetic construct
  REGION 1..122: note = Synthetic
EVQLVESGGGLVQPGGSLRLSCAASGFTFSTYSMHWVRQAPGKGLEYVSTINNNGDTTYYADSVKGRFTISRDNSKNTLYLQLGSLRPEDMAVYYCARQTYTSSWYGGFDSWGQGTLVTVSS

SEQ ID NO: 211 - DNA, 24 bp, synthetic construct
  misc_feature 1..24: note = Synthetic
  source 1..24: mol_type = other DNA
ggattcaccttcagtacctattct

SEQ ID NO: 212 - protein, 8 aa, synthetic construct
  REGION 1..8: note = Synthetic
GFTFSTYS

SEQ ID NO: 213 - DNA, 24 bp, synthetic construct
  misc_feature 1..24: note = Synthetic
  source 1..24: mol_type = other DNA
attaataataatggggataccaca

SEQ ID NO: 214 - protein, 8 aa, synthetic construct
  REGION 1..8: note = Synthetic
INNNGDTT

SEQ ID NO: 215 - DNA, 45 bp, synthetic construct
  misc_feature 1..45: note = Synthetic
  source 1..45: mol_type = other DNA
gcgagacagacgtataccagcagctggtacggggggttcgactcc

SEQ ID NO: 216 - protein, 15 aa, synthetic construct
  REGION 1..15: note = Synthetic
ARQTYTSSWYGGFDS

SEQ ID NO: 217 - DNA, 321 bp, synthetic construct
  misc_feature 1..321: note = Synthetic
  source 1..321: mol_type = other DNA
gacatccagatgacccagtctccatcttccgtgtctgcatctgtaggcgacagagtcaccatcacttgtcgggcgagtcagggtattaccagctggttagcctggtatcagcagaaaccagggaaagcccctaaactcctgatctatgctgcatccaatttgcaaagtggggtcccatcaaggttcagcggcagtggatctgggacagatttcactctcaccatcaccagcctgcagcctgaggattttgcaacttactattgtcaacaggctaacagtctcccattcactttcggccctgggaccaaagtggatatcaaa

SEQ ID NO: 218 - protein, 107 aa, synthetic construct
  REGION 1..107: note = Synthetic
DIQMTQSPSSVSASVGDRVTITCRASQGITSWLAWYQQKPGKAPKLLIYAASNLQSGVPSRFSGSGSGTDFTLTITSLQPEDFATYYCQQANSLPFTFGPGTKVDIK

SEQ ID NO: 219 - DNA, 18 bp, synthetic construct
  misc_feature 1..18: note = Synthetic
  source 1..18: mol_type = other DNA
cagggtattaccagctgg

SEQ ID NO: 220 - protein, 6 aa, synthetic construct
  REGION 1..6: note = Synthetic
QGITSW

SEQ ID NO: 221-222 - skipped (2 entries)

SEQ ID NO: 223 - DNA, 27 bp, synthetic construct
  misc_feature 1..27: note = Synthetic
  source 1..27: mol_type = other DNA
caacaggctaacagtctcccattcact

SEQ ID NO: 224 - protein, 9 aa, synthetic construct
  REGION 1..9: note = Synthetic
QQANSLPFT

SEQ ID NO: 225 - DNA, 366 bp, synthetic construct
  misc_feature 1..366: note = Synthetic
  source 1..366: mol_type = other DNA
gaggtgcagctggtggagtctgggggaggcttggtacagcctggggggtccctgagactctcctgtgcagcctctggattcacccttagcagctatgccatgagctgggtccgccaggctccagggaaggggctggagtgggtctcagctattagtggtagtggtggcagcacatactacgcagactccgtgaagggccggttcaccatctccagagacaattccaagaactcgctgtatctgcaattgaacagcctgagagccgaggacacggccgtatattactgtgcgaagacgctgtatactaccagctggtacgggggcttccagcactggggccagggcaccctggtcactgtctcctca

SEQ ID NO: 226 - protein, 122 aa, synthetic construct
  REGION 1..122: note = Synthetic
EVQLVESGGGLVQPGGSLRLSCAASGFTLSSYAMSWVRQAPGKGLEWVSAISGSGGSTYYADSVKGRFTISRDNSKNSLYLQLNSLRAEDTAVYYCAKTLYTTSWYGGFQHWGQGTLVTVSS

SEQ ID NO: 227 - DNA, 24 bp, synthetic construct
  misc_feature 1..24: note = Synthetic
  source 1..24: mol_type = other DNA
ggattcacccttagcagctatgcc

SEQ ID NO: 228 - protein, 8 aa, synthetic construct
  REGION 1..8: note = Synthetic
GFTLSSYA

SEQ ID NO: 229 - DNA, 24 bp, synthetic construct
  misc_feature 1..24: note = Synthetic
  source 1..24: mol_type = other DNA
attagtggtagtggtggcagcaca

SEQ ID NO: 230 - protein, 8 aa, synthetic construct
  REGION 1..8: note = Synthetic
ISGSGGST

SEQ ID NO: 231 - DNA, 45 bp, synthetic construct
  misc_feature 1..45: note = Synthetic
  source 1..45: mol_type = other DNA
gcgaagacgctgtatactaccagctggtacgggggcttccagcac

SEQ ID NO: 232 - protein, 15 aa, synthetic construct
  REGION 1..15: note = Synthetic
AKTLYTTSWYGGFQH

SEQ ID NO: 233 - DNA, 321 bp, synthetic construct
  misc_feature 1..321: note = Synthetic
  source 1..321: mol_type = other DNA
gacatccagatgacccagtctccatcttccgtgtctgcatctataggagacagagtcaccatcacttgtcgggcgagtcagggaatcagcagttggttagcctggtatcagcagaaaccagggaaagtccctaagctcctgatctatgctgcgtcctctttgcaaagtgggttcccatcaaggttcagcggcagtggatctgggacagatttcactctcaccatcagtagcctgcagcccgaagattttgcaacttactattgtcaacagactcacagtttcccgtggacggtcggccaagggaccaaggtggaaatcaaa

SEQ ID NO: 234 - protein, 107 aa, synthetic construct
  REGION 1..107: note = Synthetic
DIQMTQSPSSVSASIGDRVTITCRASQGISSWLAWYQQKPGKVPKLLIYAASSLQSGFPSRFSGSGSGTDFTLTISSLQPEDFATYYCQQTHSFPWTVGQGTKVEIK

SEQ ID NO: 235 - DNA, 18 bp, synthetic construct
  misc_feature 1..18: note = Synthetic
  source 1..18: mol_type = other DNA
cagggaatcagcagttgg

SEQ ID NO: 236 - protein, 6 aa, synthetic construct
  REGION 1..6: note = Synthetic
QGISSW

SEQ ID NO: 237-238 - skipped (2 entries)

SEQ ID NO: 239 - DNA, 24 bp, synthetic construct
  misc_feature 1..24: note = Synthetic
  source 1..24: mol_type = other DNA
caacagactcacagtttcccgtgg

SEQ ID NO: 240 - protein, 8 aa, synthetic construct
  REGION 1..8: note = Synthetic
QQTHSFPW

SEQ ID NO: 241 - DNA, 366 bp, synthetic construct
  misc_feature 1..366: note = Synthetic
  source 1..366: mol_type = other DNA
gaggtgcagctggtggagtctgggggaggcttggtacagcctggggggtccctgagactctcctgtgcagcctctggattcacccttaggagctatttcatgacctgggtccgccaggttccagggaaggggctggagggggtctcagctattagtggcattagtggtggcacatactacacagactccgttaagggccggttcaccatctccagagacaattccaagaacacgctgtttctgcaaatgaacagcctgagagccgaggacacggccgtatatttctgtgcgagaacggtgtatagtagtagttactacgggggcttccagcactggggccagggcaccctggtcaccgtctcctca

SEQ ID NO: 242 - protein, 122 aa, synthetic construct
  REGION 1..122: note = Synthetic
EVQLVESGGGLVQPGGSLRLSCAASGFTLRSYFMTWVRQVPGKGLEGVSAISGISGGTYYTDSVKGRFTISRDNSKNTLFLQMNSLRAEDTAVYFCARTVYSSSYYGGFQHWGQGTLVTVSS

SEQ ID NO: 243 - DNA, 24 bp, synthetic construct
  misc_feature 1..24: note = Synthetic
  source 1..24: mol_type = other DNA
ggattcacccttaggagctatttc

SEQ ID NO: 244 - protein, 8 aa, synthetic construct
  REGION 1..8: note = Synthetic
GFTLRSYF

SEQ ID NO: 245 - DNA, 24 bp, synthetic construct
  misc_feature 1..24: note = Synthetic
  source 1..24: mol_type = other DNA
attagtggcattagtggtggcaca

SEQ ID NO: 246 - protein, 8 aa, synthetic construct
  REGION 1..8: note = Synthetic
ISGISGGT

SEQ ID NO: 247 - DNA, 45 bp, synthetic construct
  misc_feature 1..45: note = Synthetic
  source 1..45: mol_type = other DNA
gcgagaacggtgtatagtagtagttactacgggggcttccagcac

SEQ ID NO: 248 - protein, 15 aa, synthetic construct
  REGION 1..15: note = Synthetic
ARTVYSSSYYGGFQH

SEQ ID NO: 249 - DNA, 321 bp, synthetic construct
  misc_feature 1..321: note = Synthetic
  source 1..321: mol_type = other DNA
gacatccagatgacccagtctccatcttccgtgtctgtatctgtaggagacagagtcaccatcacttgtcgggcgagtcagggtattagcagttggttagcctggtatcagcagaaaccagggaaagcccctaagctcctgatctatgttgcatccagtttacaaagtggggtcccatcaaggttcagcggcagtggatctgggacagatttcactctcaccatcagcagcctgcagcctgaagattttgcaacttactattgtcaacagactaacagtttccctctcactttcggcggagggaccaaggtggagatcaaa

SEQ ID NO: 250 - protein, 107 aa, synthetic construct
  REGION 1..107: note = Synthetic
DIQMTQSPSSVSVSVGDRVTITCRASQGISSWLAWYQQKPGKAPKLLIYVASSLQSGVPSRFSGSGSGTDFTLTISSLQPEDFATYYCQQTNSFPLTFGGGTKVEIK

SEQ ID NO: 251 - DNA, 18 bp, synthetic construct
  misc_feature 1..18: note = Synthetic
  source 1..18: mol_type = other DNA
cagggtattagcagttgg

SEQ ID NO: 252 - protein, 6 aa, synthetic construct
  REGION 1..6: note = Synthetic
QGISSW

SEQ ID NO: 253-254 - skipped (2 entries)

SEQ ID NO: 255 - DNA, 27 bp, synthetic construct
  misc_feature 1..27: note = Synthetic
  source 1..27: mol_type = other DNA
caacagactaacagtttccctctcact

SEQ ID NO: 256 - protein, 9 aa, synthetic construct
  REGION 1..9: note = Synthetic
QQTNSFPLT

SEQ ID NO: 257 - DNA, 366 bp, synthetic construct
  misc_feature 1..366: note = Synthetic
  source 1..366: mol_type = other DNA
gaggtgcagctggtggagtctgggggaggcttggtacagcctggggggtccctgagactctcctgtgcagcctctggattcacccttaggagttatgtcatgtactgggtccgccagggtccagggaaggggctggagggggtctcaggtattagtggcagtagtggtggcacatactacacagactccgtgaagggccggttcaccatctccagagacaattccaagaacacgctgtttctgcaaatgaacagcctgagagccgaggacacggccgtatatttctgtgcgagatcggtgtatagtaccacctggtacgggggcttccagcactggggccagggcaccctggtcaccgtctcctca

SEQ ID NO: 258 - protein, 122 aa, synthetic construct
  REGION 1..122: note = Synthetic
EVQLVESGGGLVQPGGSLRLSCAASGFTLRSYVMYWVRQGPGKGLEGVSGISGSSGGTYYTDSVKGRFTISRDNSKNTLFLQMNSLRAEDTAVYFCARSVYSTTWYGGFQHWGQGTLVTVSS

SEQ ID NO: 259 - DNA, 24 bp, synthetic construct
  misc_feature 1..24: note = Synthetic
  source 1..24: mol_type = other DNA
ggattcacccttaggagttatgtc

SEQ ID NO: 260 - protein, 8 aa, synthetic construct
  REGION 1..8: note = Synthetic
GFTLRSYV

SEQ ID NO: 261 - DNA, 24 bp, synthetic construct
  misc_feature 1..24: note = Synthetic
  source 1..24: mol_type = other DNA
attagtggcagtagtggtggcaca

SEQ ID NO: 262 - protein, 8 aa, synthetic construct
  REGION 1..8: note = Synthetic
ISGSSGGT

SEQ ID NO: 263 - DNA, 45 bp, synthetic construct
  misc_feature 1..45: note = Synthetic
  source 1..45: mol_type = other DNA
gcgagatcggtgtatagtaccacctggtacgggggcttccagcac

SEQ ID NO: 264 - protein, 15 aa, synthetic construct
  REGION 1..15: note = Synthetic
ARSVYSTTWYGGFQH

SEQ ID NO: 265 - DNA, 321 bp, synthetic construct
  misc_feature 1..321: note = Synthetic
  source 1..321: mol_type = other DNA
gacatccagatgacccagtctccatcttccgtgtctgtatctgtgggagacagagtcaccatcacttgtcgggcgagtcaggttattagcagttggttagcctggtatcagctgaaaccagggaaagcccctaaactcctgatctatgctgcatccagtttacaaagtggggtcccatcaaggttcagcggcagtggatctgggacagatttcactctcaccatcagcggcctgcagcctgaagattttgcagtttactattgtcaacagactaacagtttccctctcactttcggcggagggaccaaggtggagatcaaa

SEQ ID NO: 266 - protein, 107 aa, synthetic construct
  REGION 1..107: note = Synthetic
DIQMTQSPSSVSVSVGDRVTITCRASQVISSWLAWYQLKPGKAPKLLIYAASSLQSGVPSRFSGSGSGTDFTLTISGLQPEDFAVYYCQQTNSFPLTFGGGTKVEIK

SEQ ID NO: 267 - DNA, 18 bp, synthetic construct
  misc_feature 1..18: note = Synthetic
  source 1..18: mol_type = other DNA
caggttattagcagttgg

SEQ ID NO: 268 - protein, 6 aa, synthetic construct
  REGION 1..6: note = Synthetic
QVISSW

SEQ ID NO: 269-270 - skipped (2 entries)

SEQ ID NO: 271 - DNA, 27 bp, synthetic construct
  misc_feature 1..27: note = Synthetic
  source 1..27: mol_type = other DNA
caacagactaacagtttccctctcact

SEQ ID NO: 272 - protein, 9 aa, synthetic construct
  REGION 1..9: note = Synthetic
QQTNSFPLT

SEQ ID NO: 273 - DNA, 366 bp, synthetic construct
  misc_feature 1..366: note = Synthetic
  source 1..366: mol_type = other DNA
gaggtgcagctggtggagtctgggggaaacttggaacagcctggggggtcccttagactctcctgtacagcctctggattcacctttagcagatctgccatgaactgggtccgccgggctccagggaaggggctggagtgggtctcaggaattagtggtagtggtggtcgaacatactacgcagactccgtgaagggccggttcaccatctccagagacaattccaagaatacgctatatctgcaaatgaacagcctgagcgccgaggacacggccgcatattactgtgcgaaagattcgtatactaccagttggtacggaggtatggacgtctggggccacgggaccacggtcaccgtctcctca

SEQ ID NO: 274 - protein, 122 aa, synthetic construct
  REGION 1..122: note = Synthetic
EVQLVESGGNLEQPGGSLRLSCTASGFTFSRSAMNWVRRAPGKGLEWVSGISGSGGRTYYADSVKGRFTISRDNSKNTLYLQMNSLSAEDTAAYYCAKDSYTTSWYGGMDVWGHGTTVTVSS

SEQ ID NO: 275 - DNA, 24 bp, synthetic construct
  misc_feature 1..24: note = Synthetic
  source 1..24: mol_type = other DNA
ggattcacctttagcagatctgcc

SEQ ID NO: 276 - protein, 8 aa, synthetic construct
  REGION 1..8: note = Synthetic
GFTFSRSA

SEQ ID NO: 277 - DNA, 24 bp, synthetic construct
  misc_feature 1..24: note = Synthetic
  source 1..24: mol_type = other DNA
attagtggtagtggtggtcgaaca

SEQ ID NO: 278 - protein, 8 aa, synthetic construct
  REGION 1..8: note = Synthetic
ISGSGGRT

SEQ ID NO: 279 - DNA, 45 bp, synthetic construct
  misc_feature 1..45: note = Synthetic
  source 1..45: mol_type = other DNA
gcgaaagattcgtatactaccagttggtacggaggtatggacgtc

SEQ ID NO: 280 - protein, 15 aa, synthetic construct
  REGION 1..15: note = Synthetic
AKDSYTTSWYGGMDV

SEQ ID NO: 281 - DNA, 321 bp, synthetic construct
  misc_feature 1..321: note = Synthetic
  source 1..321: mol_type = other DNA
gacatccagatgacccagtctccatcttccgtgtctgcatctgtaggagacagagtcaccatcacttgtcgggcgagtcagggtattttcagctggttagcctggtatcagcagaaaccaggaaaagcccctaagctcctgatctatgctgcttccagtttacaaagtggggtcccatcaagattcagcggcagtggatctgggacagatttcactctcaccatcagcagcctgcagcctgaggattttgcaatttactattgtcaacaggctaacagtgtcccgatcaccttcggccaagggacacgactggagattaaa

SEQ ID NO: 282 - protein, 107 aa, synthetic construct
  REGION 1..107: note = Synthetic
DIQMTQSPSSVSASVGDRVTITCRASQGIFSWLAWYQQKPGKAPKLLIYAASSLQSGVPSRFSGSGSGTDFTLTISSLQPEDFAIYYCQQANSVPITFGQGTRLEIK

SEQ ID NO: 283 - DNA, 18 bp, synthetic construct
  misc_feature 1..18: note = Synthetic
  source 1..18: mol_type = other DNA
cagggtattttcagctgg

SEQ ID NO: 284 - protein, 6 aa, synthetic construct
  REGION 1..6: note = Synthetic
QGIFSW

SEQ ID NO: 285-286 - skipped (2 entries)

SEQ ID NO: 287 - DNA, 27 bp, synthetic construct
  misc_feature 1..27: note = Synthetic
  source 1..27: mol_type = other DNA
caacaggctaacagtgtcccgatcacc

SEQ ID NO: 288 - protein, 9 aa, synthetic construct
  REGION 1..9: note = Synthetic
QQANSVPIT

SEQ ID NO: 289 - DNA, 366 bp, synthetic construct
  misc_feature 1..366: note = Synthetic
  source 1..366: mol_type = other DNA
gaggtgcagctggtggagtctgggggaggcttggtacagcctggggggtccctgagactctcctgttcagcctctggattcacctttagcagctatgccatgaactgggtccgccaggctccagggaaggggctggagtgggtcaccgctattagtggcagtggtggtggcacatactacgcagactccgtgaagggccggttcaccatctccagagacaattccaagaactcgctgtttctgcaattgaacagcctgagagccgaggacacggccgtgtattactgtgcgaaacaaacgtataccagcagctggtacggtggctttgatatctggggccaggggacaatggtcaccgtctcttca

SEQ ID NO: 290 - protein, 122 aa, synthetic construct
  REGION 1..122: note = Synthetic
EVQLVESGGGLVQPGGSLRLSCSASGFTFSSYAMNWVRQAPGKGLEWVTAISGSGGGTYYADSVKGRFTISRDNSKNSLFLQLNSLRAEDTAVYYCAKQTYTSSWYGGFDIWGQGTMVTVSS

SEQ ID NO: 291 - DNA, 24 bp, synthetic construct
  misc_feature 1..24: note = Synthetic
  source 1..24: mol_type = other DNA
ggattcacctttagcagctatgcc

SEQ ID NO: 292 - protein, 8 aa, synthetic construct
  REGION 1..8: note = Synthetic
GFTFSSYA

SEQ ID NO: 293 - DNA, 24 bp, synthetic construct
  misc_feature 1..24: note = Synthetic
  source 1..24: mol_type = other DNA
attagtggcagtggtggtggcaca

SEQ ID NO: 294 - protein, 8 aa, synthetic construct
  REGION 1..8: note = Synthetic
ISGSGGGT

SEQ ID NO: 295 - DNA, 45 bp, synthetic construct
  misc_feature 1..45: note = Synthetic
  source 1..45: mol_type = other DNA
gcgaaacaaacgtataccagcagctggtacggtggctttgatatc

SEQ ID NO: 296 - protein, 15 aa, synthetic construct
  REGION 1..15: note = Synthetic
AKQTYTSSWYGGFDI

SEQ ID NO: 297 - DNA, 321 bp, synthetic construct
  misc_feature 1..321: note = Synthetic
  source 1..321: mol_type = other DNA
gacatccagatgacccagtcgccatcttccgtgtccgcgtctgtaggagacagagtcaccatcacttgtcgggcgagtcagggttttagttcctggttagcctggtatcagcagataccagggaaagcccccaagctcctgatctatgctgcatcaaggttgcaaagtggggtcccatccaggttccgcggcagtggatctgggacagatttcactctcaccatcagcagcctgcagcctgaggattttgcaacttactattgtcaacaggctaacagtttcccgctcactttcggcggagggaccaaggtggagatcaaa

SEQ ID NO: 298 - protein, 107 aa, synthetic construct
  REGION 1..107: note = Synthetic
DIQMTQSPSSVSASVGDRVTITCRASQGFSSWLAWYQQIPGKAPKLLIYAASRLQSGVPSRFRGSGSGTDFTLTISSLQPEDFATYYCQQANSFPLTFGGGTKVEIK

SEQ ID NO: 299 - DNA, 18 bp, synthetic construct
  misc_feature 1..18: note = Synthetic
  source 1..18: mol_type = other DNA
cagggttttagttcctgg

SEQ ID NO: 300 - protein, 6 aa, synthetic construct
  REGION 1..6: note = Synthetic
QGFSSW

SEQ ID NO: 301-302 - skipped (2 entries)

SEQ ID NO: 303 - DNA, 27 bp, synthetic construct
  misc_feature 1..27: note = Synthetic
  source 1..27: mol_type = other DNA
caacaggctaacagtttcccgctcact

SEQ ID NO: 304 - protein, 9 aa, synthetic construct
  REGION 1..9: note = Synthetic
QQANSFPLT

SEQ ID NO: 305 - protein, 167 aa, synthetic construct
  REGION 1..167: note = Synthetic
SITGISPITESLASLSTYNDQSITFALEDESYEIYVEDLKKDKKKDKVLLSYYESQHPSSESGDGVDGKMLMVTLSPTKDFWLQANNKEHSVELHKCEKPLPDQAFFVLHNRSFNCVSFECKTDPGVFIGVKDNHLALIKVDYSENLGSENILFKLSEILEHHHHHH

SEQ ID NO: 306 - protein, 167 aa, synthetic construct; identical to SEQ ID NO: 305
  REGION 1..167: note = Synthetic

SEQ ID NO: 307 - DNA, 354 bp, synthetic construct
  misc_feature 1..354: note = Synthetic
  source 1..354: mol_type = other DNA
caggtcaccttgaaggagtctggtcctgtgctggtgaaacccacagagagcctcacgctgacctgctccgtctctggattctcactcagtaatgttagaatgggtgtgagctggatccgtcagtccccagggaaggccctggagtggcttgcacacattttttcgaatgacgaaaaatcctacaccacatctctgaagaccaggctcaccatctccaaggacacctccagaagccaggtggtccttaccatgaccgacatggaccctggggacacagccacatattactgtgcacggatacggaatttggcctttaattactggggccagggaaccctggtcaccgtctcctca

SEQ ID NO: 308 - protein, 118 aa, synthetic construct
  REGION 1..118: note = Synthetic
QVTLKESGPVLVKPTESLTLTCSVSGFSLSNVRMGVSWIRQSPGKALEWLAHIFSNDEKSYTTSLKTRLTISKDTSRSQVVLTMTDMDPGDTATYYCARIRNLAFNYWGQGTLVTVSS

SEQ ID NO: 309 - DNA, 30 bp, synthetic construct
  misc_feature 1..30: note = Synthetic
  source 1..30: mol_type = other DNA
ggattctcactcagtaatgttagaatgggt

SEQ ID NO: 310 - protein, 10 aa, synthetic construct
  REGION 1..10: note = Synthetic
GFSLSNVRMG

SEQ ID NO: 311 - DNA, 21 bp, synthetic construct
  misc_feature 1..21: note = Synthetic
  source 1..21: mol_type = other DNA
attttttcgaatgacgaaaaa

SEQ ID NO: 312 - protein, 7 aa, synthetic construct
  REGION 1..7: note = Synthetic
IFSNDEK

SEQ ID NO: 313 - DNA, 30 bp, synthetic construct
  misc_feature 1..30: note = Synthetic
  source 1..30: mol_type = other DNA
gcacggatacggaatttggcctttaattac

SEQ ID NO: 314 - protein, 10 aa, synthetic construct
  REGION 1..10: note = Synthetic
ARIRNLAFNY

SEQ ID NO: 315 - DNA, 339 bp, synthetic construct
  misc_feature 1..339: note = Synthetic
  source 1..339: mol_type = other DNA
gacttcgtgatgacccagtctccagactccctggctgtgtctctgggcgagagggccaccatcaactgcaagtccagccagagtgtgttacacaggtccagcaataagaactacttagcttggtatcagcagaagccaggacagcctcctaacctgctcatttactgggcatctacccgggaatccggggtccctgaccgattcagtggcagcgggtctgggacagatttcactctcaccatcagcagcctgcaggctgaagatgtggcagtttattactgtcagcaatattatggtactctatttactttcggccctgggaccaaagtggatatcaaa

SEQ ID NO: 316 - protein, 113 aa, synthetic construct
  REGION 1..113: note = Synthetic
DFVMTQSPDSLAVSLGERATINCKSSQSVLHRSSNKNYLAWYQQKPGQPPNLLIYWASTRESGVPDRFSGSGSGTDFTLTISSLQAEDVAVYYCQQYYGTLFTFGPGTKVDIK

SEQ ID NO: 317 - DNA, 36 bp, synthetic construct
  misc_feature 1..36: note = Synthetic
  source 1..36: mol_type = other DNA
cagagtgtgttacacaggtccagcaataagaactac

SEQ ID NO: 318 - protein, 12 aa, synthetic construct
  REGION 1..12: note = Synthetic
QSVLHRSSNKNY

SEQ ID NO: 319-320 - skipped (2 entries)

SEQ ID NO: 321 - DNA, 27 bp, synthetic construct
  misc_feature 1..27: note = Synthetic
  source 1..27: mol_type = other DNA
cagcaatattatggtactctatttact

SEQ ID NO: 322 - protein, 9 aa, synthetic construct
  REGION 1..9: note = Synthetic
QQYYGTLFT

SEQ ID NO: 323 - protein, 537 aa, synthetic construct
  REGION 1..537: note = hST2-hFc
KFSKQSWGLENEALIVRCPRQGKPSYTVDWYYSQTNKSIPTQERNRVFASGQLLKFLPAAVADSGIYTCIVRSPTFNRTGYANVTIYKKQSDCNVPDYLMYSTVSGSEKNSKIYCPTIDLYNWTAPLEWFKNCQALQGSRYRAHKSFLVIDNVMTEDAGDYTCKFIHNENGANYSVTATRSFTVKDEQGFSLFPVIGAPAQNEIKEVEIGKNANLTCSACFGKGTQFLAAVLWQLNGTKITDFGEPRIQQEEGQNQSFSNGLACLDMVLRIADVKEEDLLLQYDCLALNLHGLRRHTVRLSRKNPIDHHSDKTHTCPPCPAPELLGGPSVFLFPPKPKDTLMISRTPEVTCVVVDVSHEDPEVKFNWYVDGVEVHNAKTKPREEQYNSTYRVVSVLTVLHQDWLNGKEYKCKVSNKALPAPIEKTISKAKGQPREPQVYTLPPSRDELTKNQVSLTCLVKGFYPSDIAVEWESNGQPENNYKTTPPVLDSDGSFFLYSKLTVDKSRWQQGNVFSCSVMHEALHNHYTQKSLSLSPGK

SEQ ID NO: 324 - protein, 543 aa, synthetic construct
  REGION 1..543: note = hST2-mFc
KFSKQSWGLENEALIVRCPRQGKPSYTVDWYYSQTNKSIPTQERNRVFASGQLLKFLPAAVADSGIYTCIVRSPTFNRTGYANVTIYKKQSDCNVPDYLMYSTVSGSEKNSKIYCPTIDLYNWTAPLEWFKNCQALQGSRYRAHKSFLVIDNVMTEDAGDYTCKFIHNENGANYSVTATRSFTVKDEQGFSLFPVIGAPAQNEIKEVEIGKNANLTCSACFGKGTQFLAAVLWQLNGTKITDFGEPRIQQEEGQNQSFSNGLACLDMVLRIADVKEEDLLLQYDCLALNLHGLRRHTVRLSRKNPIDHHSEPRGPTIKPCPPCKCPAPNLLGGPSVFIFPPKIKDVLMISLSPIVTCVVVDVSEDDPDVQISWFVNNVEVHTAQTQTHREDYNSTLRVVSALPIQHQDWMSGKEFKCKVNNKDLPAPIERTISKPKGSVRAPQVYVLPPPEEEMTKKQVTLTCMVTDFMPEDIYVEWTNNGKTELNYKNTEPVLDSDGSYFMYSKLRVEKKNWVERNSYSCSVVHEGLHNHHTTKSFSRTPGK

SEQ ID NO: 325 - protein, 884 aa, synthetic construct
  REGION 1..884: note = hST2-hIL1RAcP-mFc
KFSKQSWGLENEALIVRCPRQGKPSYTVDWYYSQTNKSIPTQERNRVFASGQLLKFLPAAVADSGIYTCIVRSPTFNRTGYANVTIYKKQSDCNVPDYLMYSTVSGSEKNSKIYCPTIDLYNWTAPLEWFKNCQALQGSRYRAHKSFLVIDNVMTEDAGDYTCKFIHNENGANYSVTATRSFTVKDEQGFSLFPVIGAPAQNEIKEVEIGKNANLTCSACFGKGTQFLAAVLWQLNGTKITDFGEPRIQQEEGQNQSFSNGLACLDMVLRIADVKEEDLLLQYDCLALNLHGLRRHTVRLSRKNPIDHHSSERCDDWGLDTMRQIQVFEDEPARIKCPLFEHFLKFNYSTAHSAGLTLIWYWTRQDRDLEEPINFRLPENRISKEKDVLWFRPTLLNDTGNYTCMLRNTTYCSKVAFPLEVVQKDSCFNSPMKLPVHKLYIEYGIQRITCPNVDGYFPSSVKPTITWYMGCYKIQNFNNVIPEGMNLSFLIALISNNGNYTCVVTYPENGRTFHLTRTLTVKVVGSPKNAVPPVIHSPNDHVVYEKEPGEELLIPCTVYFSFLMDSRNEVWWTIDGKKPDDITIDVTINESISHSRTEDETRTQILSIKKVTSEDLKRSYVCHARSAKGEVAKAAKVKQKVPAPRYTVESGEPRGPTIKPCPPCKCPAPNLLGGPSVFIFPPKIKDVLMISLSPIVTCVVVDVSEDDPDVQISWFVNNVEVHTAQTQTHREDYNSTLRVVSALPIQHQDWMSGKEFKCKVNNKDLPAPIERTISKPKGSVRAPQVYVLPPPEEEMTKKQVTLTCMVTDFMPEDIYVEWTNNGKTELNYKNTEPVLDSDGSYFMYSKLRVEKKNWVERNSYSCSVVHEGLHNHHTTKSFSRTPGK

SEQ ID NO: 326 - protein, 880 aa, synthetic construct
  REGION 1..880: note = mST2-mIL1RAcP-mFc
SKSSWGLENEALIVRCPQRGRSTYPVEWYYSDTNESIPTQKRNRIFVSRDRLKFLPARVEDSGIYACVIRSPNLNKTGYLNVTIHKKPPSCNIPDYLMYSTVRGSDKNFKITCPTIDLYNWTAPVQWFKNCKALQEPRFRAHRSYLFIDNVTHDDEGDYTCQFTHAENGTNYIVTATRSFTVEEKGFSMFPVITNPPYNHTMEVEIGKPASIACSACFGKGSHFLADVLWQINKTVVGNFGEARIQEEEGRNESSSNDMDCLTSVLRITGVTEKDLSLEYDCLALNLHGMIRHTIRLRRKQPIDHRSERCDDWGLDTMRQIQVFEDEPARIKCPLFEHFLKYNYSTAHSSGLTLIWYWTRQDRDLEEPINFRLPENRISKEKDVLWFRPTLLNDTGNYTCMLRNTTYCSKVAFPLEVVQKDSCFNSAMRFPVHKMYIEHGIHKITCPNVDGYFPSSVKPSVTWYKGCTEIVDFHNVLPEGMNLSFFIPLVSNNGNYTCVVTYPENGRLFHLTRTVTVKVVGSPKDALPPQIYSPNDRVVYEKEPGEELVIPCKVYFSFIMDSHNEVWWTIDGKKPDDVTVDITINESVSYSSTEDETRTQILSIKKVTPEDLRRNYVCHARNTKGEAEQAAKVKQKVIPPRYTVESGEPRGPTIKPCPPCKCPAPNLLGGPSVFIFPPKIKDVLMISLSPIVTCVVVDVSEDDPDVQISWFVNNVEVHTAQTQTHREDYNSTLRVVSALPIQHQDWMSGKEFKCKVNNKDLPAPIERTISKPKGSVRAPQVYVLPPPEEEMTKKQVTLTCMVTDFMPEDIYVEWTNNGKTELNYKNTEPVLDSDGSYFMYSKLRVEKKNWVERNSYSCSVVHEGLHNHHTTKSFSRTPGK

SEQ ID NO: 327 - protein, 876 aa, synthetic construct
  REGION 1..876: note = hST2-hL1RAcP-hFc
KFSKQSWGLENEALIVRCPRQGKPSYTVDWYYSQTNKSIPTQERNRVFASGQLLKFLPAAVADSGIYTCIVRSPTFNRTGYANVTIYKKQSDCNVPDYLMYSTVSGSEKNSKIYCPTIDLYNWTAPLEWFKNCQALQGSRYRAHKSFLVIDNVMTEDAGDYTCKFIHNENGANYSVTATRSFTVKDEQGFSLFPVIGAPAQNEIKEVEIGKNANLTCSACFGKGTQFLAAVLWQLNGTKITDFGEPRIQQEEGQNQSFSNGLACLDMVLRIADVKEEDLLLQYDCLALNLHGLRRHTVRLSRKNPIDHHSSERCDDWGLDTMRQIQVFEDEPARIKCPLFEHFLKFNYSTAHSAGLTLIWYWTRQDRDLEEPINFRLPENRISKEKDVLWFRPTLLNDTGNYTCMLRNTTYCSKVAFPLEVVQKDSCFNSPMKLPVHKLYIEYGIQRITCPNVDGYFPSSVKPTITWYMGCYKIQNFNNVIPEGMNLSFLIALISNNGNYTCVVTYPENGRTFHLTRTLTVKVVGSPKNAVPPVIHSPNDHVVYEKEPGEELLIPCTVYFSFLMDSRNEVWWTIDGKKPDDITIDVTINESISHSRTEDETRTQILSIKKVTSEDLKRSYVCHARSAKGEVAKAAKVKQKVPAPRYTVEDKTHTCPPCPAPELLGGPSVFLFPPKPKDTLMISRTPEVTCVVVDVSHEDPEVKFNWYVDGVEVHNAKTKPREEQYNSTYRVVSVLTVLHQDWLNGKEYKCKVSNKALPAPIEKTISKAKGQPREPQVYTLPPSRDELTKNQVSLTCLVKGFYPSDIAVEWESNGQPENNYKTTPPVLDSDGSFFLYSKLTVDKSRWQQGNVFSCSVMHEALHNHYTQKSLSLSPGK

SEQ ID NO: 328 - protein, 310 aa, synthetic construct
  REGION 1..310: note = human ST2 extracellular domain
KFSKQSWGLENEALIVRCPRQGKPSYTVDWYYSQTNKSIPTQERNRVFASGQLLKFLPAAVADSGIYTCIVRSPTFNRTGYANVTIYKKQSDCNVPDYLMYSTVSGSEKNSKIYCPTIDLYNWTAPLEWFKNCQALQGSRYRAHKSFLVIDNVMTEDAGDYTCKFIHNENGANYSVTATRSFTVKDEQGFSLFPVIGAPAQNEIKEVEIGKNANLTCSACFGKGTQFLAAVLWQLNGTKITDFGEPRIQQEEGQNQSFSNGLACLDMVLRIADVKEEDLLLQYDCLALNLHGLRRHTVRLSRKNPIDHHS

SEQ ID NO: 329 - protein, 306 aa, synthetic construct
  REGION 1..306: note = mouse ST2 extracellular domain
SKSSWGLENEALIVRCPQRGRSTYPVEWYYSDTNESIPTQKRNRIFVSRDRLKFLPARVEDSGIYACVIRSPNLNKTGYLNVTIHKKPPSCNIPDYLMYSTVRGSDKNFKITCPTIDLYNWTAPVQWFKNCKALQEPRFRAHRSYLFIDNVTHDDEGDYTCQFTHAENGTNYIVTATRSFTVEEKGFSMFPVITNPPYNHTMEVEIGKPASIACSACFGKGSHFLADVLWQINKTVVGNFGEARIQEEEGRNESSSNDMDCLTSVLRITGVTEKDLSLEYDCLALNLHGMIRHTIRLRRKQPIDHR

SEQ ID NO: 330 - protein, 339 aa, synthetic construct
  REGION 1..339: note = human IL1RAcP extracellular domain
SERCDDWGLDTMRQIQVFEDEPARIKCPLFEHFLKFNYSTAHSAGLTLIWYWTRQDRDLEEPINFRLPENRISKEKDVLWFRPTLLNDTGNYTCMLRNTTYCSKVAFPLEVVQKDSCFNSPMKLPVHKLYIEYGIQRITCPNVDGYFPSSVKPTITWYMGCYKIQNFNNVIPEGMNLSFLIALISNNGNYTCVVTYPENGRTFHLTRTLTVKVVGSPKNAVPPVIHSPNDHVVYEKEPGEELLIPCTVYFSFLMDSRNEVWWTIDGKKPDDITIDVTINESISHSRTEDETRTQILSIKKVTSEDLKRSYVCHARSAKGEVAKAAKVKQKVPAPRYTVE

SEQ ID NO: 331 - protein, 339 aa, synthetic construct
  REGION 1..339: note = mouse IL1RAcP extracellular domain
SERCDDWGLDTMRQIQVFEDEPARIKCPLFEHFLKYNYSTAHSSGLTLIWYWTRQDRDLEEPINFRLPENRISKEKDVLWFRPTLLNDTGNYTCMLRNTTYCSKVAFPLEVVQKDSCFNSAMRFPVHKMYIEHGIHKITCPNVDGYFPSSVKPSVTWYKGCTEIVDFHNVLPEGMNLSFFIPLVSNNGNYTCVVTYPENGRLFHLTRTVTVKVVGSPKDALPPQIYSPNDRVVYEKEPGEELVIPCKVYFSFIMDSHNEVWWTIDGKKPDDVTVDITINESVSYSSTEDETRTQILSIKKVTPEDLRRNYVCHARNTKGEAEQAAKVKQKVIPPRYTVE

SEQ ID NO: 332 - protein, 227 aa, synthetic construct
  REGION 1..227: note = human IgG1 Fc
DKTHTCPPCPAPELLGGPSVFLFPPKPKDTLMISRTPEVTCVVVDVSHEDPEVKFNWYVDGVEVHNAKTKPREEQYNSTYRVVSVLTVLHQDWLNGKEYKCKVSNKALPAPIEKTISKAKGQPREPQVYTLPPSRDELTKNQVSLTCLVKGFYPSDIAVEWESNGQPENNYKTTPPVLDSDGSFFLYSKLTVDKSRWQQGNVFSCSVMHEALHNHYTQKSLSLSPGK

SEQ ID NO: 333 - protein, 233 aa, synthetic construct
  REGION 1..233: note = mouse IgG2a Fc
EPRGPTIKPCPPCKCPAPNLLGGPSVFIFPPKIKDVLMISLSPIVTCVVVDVSEDDPDVQISWFVNNVEVHTAQTQTHREDYNSTLRVVSALPIQHQDWMSGKEFKCKVNNKDLPAPIERTISKPKGSVRAPQVYVLPPPEEEMTKKQVTLTCMVTDFMPEDIYVEWTNNGKTELNYKNTEPVLDSDGSYFMYSKLRVEKKNWVERNSYSCSVVHEGLHNHHTTKSFSRTPGK

SEQ ID NO: 334 - protein, 167 aa, synthetic construct; identical to SEQ ID NO: 305
  REGION 1..167: note = M.fascicularis IL-33-6His

SEQ ID NO: 335 - protein, 117 aa, synthetic construct
  REGION 1..117: note = HCVR-mouse surrogate IL-4R Ab
EVQLQQSGPELVKPGASVRMSCKASGYTFTDYNIHWVKQSHGKSLEWIGYIYPNNGDNGYNQKFRGKATLTVDKSSSTAYMELRSLTSDDSAVYYCARGRLRYFDVWGTGTTVTVSS

SEQ ID NO: 336 - protein, 111 aa, synthetic construct
  REGION 1..111: note = LCVR-mouse surrogate IL-4R Ab
NIVLTQSPASLAVSLGQRATISCRASESVDNYGHSFMHWYQQKPGQPPKLLIYLASNLESGVPARFSGSGSRTDFTLTLDPVEADDAATYYCQQYNEDPPTFGSGTKLEIK

SEQ ID NO: 337 - protein, 124 aa, synthetic construct
  REGION 1..124: note = Dupilumab HCVR
EVQLVESGGGLEQPGGSLRLSCAGSGFTFRDYAMTWVRQAPGKGLEWVSSISGSGGNTYYADSVKGRFTISRDNSKNTLYLQMNSLRAEDTAVYYCAKDRLSITIRPRYYGLDVWGQGTTVTVS

SEQ ID NO: 338 - protein, 112 aa, synthetic construct [sequence omitted]

SEQ ID NO: 339 - protein, 8 aa, synthetic construct
  REGION 1..8: note = Dupilumab HCDR1
GFTFRDYA

SEQ ID NO: 340 - protein, 8 aa, synthetic construct
  REGION 1..8: note = Dupilumab HCDR2
ISGSGGNT

SEQ ID NO: 341 - protein, 18 aa, synthetic construct
  REGION 1..18: note = Dupilumab HCDR3
AKDRLSITIRPRYYGLDV

SEQ ID NO: 342 - protein, 11 aa, synthetic construct
  REGION 1..11: note = Dupilumab LCDR1
QSLLYSIGYNY

SEQ ID NO: 343 - skipped

SEQ ID NO: 344 - protein, 9 aa, synthetic construct
  REGION 1..9: note = Dupilumab LCDR3
MQALQTPYT

SEQ ID NO: 345 - protein, 451 aa, synthetic construct
  REGION 1..451: note = Dupilumab heavy chain
EVQLVESGGGLEQPGGSLRLSCAGSGFTFRDYAMTWVRQAPGKGLEWVSSISGSGGNTYYADSVKGRFTISRDNSKNTLYLQMNSLRAEDTAVYYCAKDRLSITIRPRYYGLDVWGQGTTVTVSSASTKGPSVFPLAPCSRSTSESTAALGCLVKDYFPEPVTVSWNSGALTSGVHTFPAVLQSSGLYSLSSVVTVPSSSLGTKTYTCNVDHKPSNTKVDKRVESKYGPPCPPCPAPEFLGGPSVFLFPPKPKDTLMISRTPEVTCVVVDVSQEDPEVQFNWYVDGVEVHNAKTKPREEQFNSTYRVVSVLTVLHQDWLNGKEYKCKVSNKGLPSSIEKTISKAKGQPREPQVYTLPPSQEEMTKNQVSLTCLVKGFYPSDIAVEWESNGQPENNYKTTPPVLDSDGSFFLYSRLTVDKSRWQEGNVFSCSVMHEALHNHYTQKSLSLSLG

SEQ ID NO: 346 - protein, 219 aa, synthetic construct
  REGION 1..219: note = Dupilumab light chain
DIVMTQSPLSLPVTPGEPASISCRSSQSLLYSIGYNYLDWYLQKSGQSPQLLIYLGSNRASGVPDRFSGSGSGTDFTLKISRVEAEDVGFYYCMQALQTPYTFGQGTKLEIKRTVAAPSVFIFPPSDEQLKSGTASVVCLLNNFYPREAKVQWKVDNALQSGNSQESVTEQDSKDSTYSLSSTLTLSKADYEKHKVYACEVTHQGLSSPVTKSFNRGEC

SEQ ID NO: 347 - protein, 207 aa, synthetic construct
  REGION 1..207: note = human IL-4Ralpha
MKVLQEPTCVSDYMSISTCEWKMNGPTNCSTELRLLYQLVFLLSEAHTCIPENNGGAGCVCHLLMDDVVSADNYTLDLWAGQQLLWKGSFKPSEHVKPRAPGNLTVHTNVSDTLLLTWSNPYPPDNYLYNHLTYAVNIWSENDPADFRIYNVTYLEPSLRIAASTLKSGISYRARVRAWAQCYNTTWSEWSPSTKWHNSYREPFEQH

SEQ ID NO: 348 - protein, 270 aa, synthetic construct
  REGION 1..270: note = hIL33_O95760 (prior to proteolytic processing)
MKPKMKYSTNKISTAKWKNTASKALCFKLGKSQQKAKEVCPMYFMKLRSGLMIKKEACYFRRETTKRPSLKTGRKHKRHLVLAACQQQSTVECFAFGISGVQKYTRALHDSSITGISPITEYLASLSTYNDQSITFALEDESYEIYVEDLKKDEKKDKVLLSYYESQHPSNESGDGVDGKMLMVTLSPTKDFWLHANNKEHSVELHKCEKPLPDQAFFVLHNMHSNCVSFECKTDPGVFIGVKDNHLALIKVDSSENLCTENILFKLSET

SEQ ID NO: 349 - protein, 159 aa, synthetic construct
  REGION 1..159: note = hIL33_mature_PEPTIDE (after proteolytic processing)
SITGISPITEYLASLSTYNDQSITFALEDESYEIYVEDLKKDEKKDKVLLSYYESQHPSNESGDGVDGKMLMVTLSPTKDFWLHANNKEHSVELHKCEKPLPDQAFFVLHNMHSNCVSFECKTDPGVFIGVKDNHLALIKVDSSENLCTENILFKLSET

SEQ ID NO: 350 - protein, 12 aa, synthetic construct
  REGION 1..12: note = Amino Acid residues 1-12 of SEQ ID NO: 349; also corresponds to residues 112-123 of SEQ ID NO: 348 (Uniprot O95760)
SITGISPITEYL

SEQ ID NO: 351 - protein, 87 aa, synthetic construct
  REGION 1..87: note = Amino Acid residues 50-94 of SEQ ID NO: 349; also corresponds to residues 161-205 of SEQ ID NO: 348 (Uniprot O95760)
ITEYLASLSTYNDQSITFALEDESYEIYVEDLKKDEKKDKVLLSYYESQHPSNESGDGVDGKMLMVTLSPTKDFWLHANNKEHSVEL

SEQ ID NO: 352 - protein, 556 aa, synthetic construct
  REGION 1..556: note = Human ST2 (See GenBank accession number NP_057316)
MGFWILAILTILMYSTAAKFSKQSWGLENEALIVRCPRQGKPSYTVDWYYSQTNKSIPTQERNRVFASGQLLKFLPAAVADSGIYTCIVRSPTFNRTGYANVTIYKKQSDCNVPDYLMYSTVSGSEKNSKIYCPTIDLYNWTAPLEWFKNCQALQGSRYRAHKSFLVIDNVMTEDAGDYTCKFIHNENGANYSVTATRSFTVKDEQGFSLFPVIGAPAQNEIKEVEIGKNANLTCSACFGKGTQFLAAVLWQLNGTKITDFGEPRIQQEEGQNQSFSNGLACLDMVLRIADVKEEDLLLQYDCLALNLHGLRRHTVRLSRKNPIDHHSIYCIIAVCSVFLMLINVLVIILKMFWIEATLLWRDIAKPYKTRNDGKLYDAYVVYPRNYKSSTDGASRVEHFVHQILPDVLENKCGYTLCIYGRDMLPGEDVVTAVETNIRKSRRHIFILTPQITHNKEFAYEQEVALHCALIQNDAKVILIEMEALSELDMLQAEALQDSLQHLMKVQGTIKWREDHIANKRSLNSKFWKHVRYQMPVPSKIPRKASSLTPLAAQKQ

SEQ ID NO: 353 - protein, 570 aa, synthetic construct
  REGION 1..570: note = Human IL-1RAcP (See GenBank accession number Q9NPH3)
MTLLWCVVSLYFYGILQSDASERCDDWGLDTMRQIQVFEDEPARIKCPLFEHFLKFNYSTAHSAGLTLIWYWTRQDRDLEEPINFRLPENRISKEKDVLWFRPTLLNDTGNYTCMLRNTTYCSKVAFPLEVVQKDSCFNSPMKLPVHKLYIEYGIQRITCPNVDGYFPSSVKPTITWYMGCYKIQNFNNVIPEGMNLSFLIALISNNGNYTCVVTYPENGRTFHLTRTLTVKVVGSPKNAVPPVIHSPNDHVVYEKEPGEELLIPCTVYFSFLMDSRNEVWWTIDGKKPDDITIDVTINESISHSRTEDETRTQILSIKKVTSEDLKRSYVCHARSAKGEVAKAAKVKQKVPAPRYTVELACGFGATVLLVVILIVVYHVYWLEMVLFYRAHFGTDETILDGKEYDIYVSYARNAEEEEFVLLTLRGVLENEFGYKLCIFDRDSLPGGIVTDETLSFIQKSRRLLVVLSPNYVLQGTQALLELKAGLENMASRGNINVILVQYKAVKETKVKELKRAKTVLTVIKWKGEKSKYPQGRFWKQLQVAMPVKKSPRRSSSDEQGLSYSSLKNV

SEQ ID NO: 354 - protein, 449 aa, synthetic construct
  REGION 1..449: note = HC OF H4H9675P
EVQLVESGGNLEQPGGSLRLSCTASGFTFSRSAMNWVRRAPGKGLEWVSGISGSGGRTYYADSVKGRFTISRDNSKNTLYLQMNSLSAEDTAAYYCAKDSYTTSWYGGMDVWGHGTTVTVSSASTKGPSVFPLAPCSRSTSESTAALGCLVKDYFPEPVTVSWNSGALTSGVHTFPAVLQSSGLYSLSSVVTVPSSSLGTKTYTCNVDHKPSNTKVDKRVESKYGPPCPPCPAPEFLGGPSVFLFPPKPKDTLMISRTPEVTCVVVDVSQEDPEVQFNWYVDGVEVHNAKTKPREEQFNSTYRVVSVLTVLHQDWLNGKEYKCKVSNKGLPSSIEKTISKAKGQPREPQVYTLPPSQEEMTKNQVSLTCLVKGFYPSDIAVEWESNGQPENNYKTTPPVLDSDGSFFLYSRLTVDKSRWQEGNVFSCSVMHEALHNHYTQKSLSLSLGK

SEQ ID NO: 355 - protein, 214 aa, synthetic construct
  REGION 1..214: note = LC OF H4H9675P
DIQMTQSPSSVSASVGDRVTITCRASQGIFSWLAWYQQKPGKAPKLLIYAASSLQSGVPSRFSGSGSGTDFTLTISSLQPEDFAIYYCQQANSVPITFGQGTRLEIKRTVAAPSVFIFPPSDEQLKSGTASVVCLLNNFYPREAKVQWKVDNALQSGNSQESVTEQDSKDSTYSLSSTLTLSKADYEKHKVYACEVTHQGLSSPVTKSFNRGEC

SEQ ID NO: 356 - protein, 166 aa, synthetic construct
  REGION 1..166: note = HUMAN IL-33 WITH HEXA-HIS TAG (AMINO ACIDS 112-270 OF GENBANK ACCESSION NO. O95760)
MSITGISPITEYLASLSTYNDQSITFALEDESYEIYVEDLKKDEKKDKVLLSYYESQHPSNESGDGVDGKMLMVTLSPTKDFWLHANNKEHSVELHKCEKPLPDQAFFVLHNMHSNCVSFECKTDPGVFIGVKDNHLALIKVDSSENLCTENILFKLSETHHHHHH

SEQ ID NO: 357 - DNA, 51 bp, synthetic construct
  misc_feature 1..51: note = Synthetic
  misc_feature 26: note = n is g or a
  source 1..51: mol_type = other DNA
tataccatcacaaagcctctcattanactttgaatccaatgagtattacta

SEQ ID NO: 358 - DNA, 51 bp, synthetic construct
  misc_feature 1..51: note = Synthetic
  misc_feature 26: note = n is g or t
  source 1..51: mol_type = other DNA
ccaatcttttctcatgaagacaccancatgacctcttattcttatttatat